European Patent Application EP 4 147 715 A1, published March 15, 2023. Title: Biofusion proteins as anti-malaria vaccines. Applicant: VAC4ALL PTE. LTD. Application EP. The sequence listing filed with the application follows.

SEQUENCE LISTING (89 sequences)

SEQ ID NO: 1 - protein, 1103 aa, Plasmodium falciparum
MSNKKRSKNENDESTSLPLENSELLIEYIHNLKSCLNVYRREIQEKNKYISIIKNDLSFHECILTNVNVVWSVFNNDLLNLLCNNEQKEEGEEIIKQRNIGDEINEYNNLTKLQNDENIKNNNMIKEDLEDDANQNILMKSPYYNIENFLQVFLKYINKKKKKVKVKVKDEGKKEKIEDKKYEQDDEEENEEEEEEEEEEEGEEENKEDEEFFKTFVSFNLYHNNNEKNISYDKNLVKQENDNKDEARGNDNMCGNYDIHNERGEMLDKGKSYSGDEKINTSDNAKSCSGDEKVITSDNGKSYDYVKNESEEQEEKENMLNNKKRSLECNPNEAKKICFSLEEKIGTVQSVKLKEYNELSKENIEKNKHDDNNICNYLSHNEGENVIEREDKLFNKLNNKNYRNEEEKKKNQINFDYLKKKIKNNQDVFEETIQKCFLINLKKTLNLINKIMYLKNVEFRKYNLDYIRKINYEKCFYYKNYIDIKKKISELQKDNESLKIQVDRLEKKKATLIYKLNNDNIRKHILDNNIKDYQNGIDNSKVSYFDEGENPYNRNNKNYRTDNKNSDDNNNNNNYYYNNYNSDDNYNSEDNEYNNGNYRFRNNYKKDSLNEDDVKKNPLKVCHKINSDSNIFVNFENIITKQNIIHSEPFRNLLKESNELYITLKEKEKENIILKNEILKMENKKDEEYEHLLNNTIEDKKELTRSIKELEINMMTCNMEKDKISNKVNTLEYEINVLKNIDKNQTMQLQQKENDILKMKLYIEKLKLSEKNLKDKIILLENEKDKMLSGIHIKDNSFNEESKSEEGKIQLRDIQNDNDEKYDDEKKRFKELFIENQKLKEELNKKRNVEEELHSLRKNYNIINEEIEEITKEFEKKQEQVDEMILQIKNKELELLDKFNNKMNKAYVEEKLKELKNTYEEKMKHINNIYKKHDDFVNIYLNLFFQARKNAILSDSQREEQMNLFIKLKDKYDIIFQKKIELTDILKNVYDCNKKLIGHCQDLEKENSTLQNKLSNEIKNSKMLSKNLSKNSDDHLLIEENNELRRRLICSVCMENFRNYIIIKCGHIYCNNCIFNNLKTRNRKCPQCKVPFDKKDLQKIFLD

SEQ ID NO: 2 - protein, 104 aa, Plasmodium falciparum
HNNNEKNISYDKNLVKQENDNKDEARGNDNMCGNYDIHNERGEMLDKGKSYSGDEKINTSDNAKSCSGDEKVITSDNGKSYDYVKNESEEQEEKENMLNNKKRS

SEQ ID NO: 3 - protein, 27 aa, Plasmodium falciparum
KKRNVEEELHSLRKNYNIINEEIEEIT

SEQ ID NO: 4 - protein, 80 aa, Plasmodium falciparum
NEEEITTKGASAQSGASAQSGASAQSGASAQSGASAQSGASAQSGTSGPSGPSGTSPSSRSNTLPRSNTSSGASPPADAS

SEQ ID NO: 5 - protein, 390 aa, Plasmodium falciparum
MAHHHHHHPGGSGSGTMAISVTMDNILSGFENEYDVIYLKPLAGVYRSLKKQIEKNIFTFNLNLNDILNSRLKKRKYFLDVLESDLMQFKHISSNEYIIEDSFKLLNSEQKNTLLKSYKYIKESVENDIKFAQEGISYYEKVLAKYKDDLESIKKVIKEEKEKFPSSPPTTPPSPAKTDEQKKESKFLPFLTNIETLYNNLVNKIDDYLINLKAKINDCNVEKDEAHVKITKLSDLKAIDDKIDLFKNPTDFEAIKKLINDDTKKDMLGKLLSTGLVQNFPNTIISKLIEGKFQDMLNISQHQCVKKQCPENSGCFRHLDEREECKCLLNYKQEGDKCVENPNPTCNENNGGCDADATCTEEDSGSSRKKITCECTKPDSYPLFDGIFCS

SEQ ID NO: 6 - protein, 272 aa, Plasmodium falciparum
MKVIKTLSIINFFIFVTFNIKNESKYSNTFINNAYNMSIRRSMAESKPSTGAGGSAGGSAGGSAGGSAGGSAGGSAGSGDGNGADAEGSSSTPATTTTTKTTTTTTTTNDAEASTSTSSENPNHKNAETNPKGKGEVQEPNQANKETQNNSNVQQDSQTKSNVPPTQDADTKSPTAQPEQAENSAPTAEQTESPELQSAPENKGTGQHGHMHGSRNNHPQNTSDSQKECTDGNKENCGAATSLLNNSSNIASINKFVVLISATLVLSFAIFI

SEQ ID NO: 7 - protein, 354 aa, Plasmodium falciparum
MKSFINITLSLFLLHLYIYINNVASKEIVKKYNLNLRNAILNNNSQIENEENVNTTITGNDFSGGEFLWPGYTEELKAKKASEDAEKAANDAENASKEAEEAAKEAVNLKESDKSYTKAKEACTAASKAKKAVETALKAKDDAEKSSKADSISTKTKEYAEKAKNAYEKAKNAYQKANQAVLKAKEASSYDYILGWEFGGGVPEHKKEENMLSHLYVSSKDKENISKENDDVLDEKEEEAEETEEEELEEKNEEETESEISEDEEEEEEEEEKEEENDKKKEQEKEQSNENNDQKKDMEAQNLISKNQNNNEKNVKEAAESIMKTLAGLIKGNNQIDSTLKDLVEELSKYFKNH

SEQ ID NO: 8 - protein, 188 aa, Plasmodium falciparum
YEKAKNAYQKANQAVLKAKEASSYDYILGWEFGGGVPEHKKEENMLSHLYVSSKDKENISKENDDVLDEKEEEAEETEEEELEEKNEEETESEISEDEEEEEEEEEKEEENDKKKEQEKEQSNENNDQKKDMEAQNLISKNQNNNEKNVKEAAESIMKTLAGLIKGNNQIDSTLKDLVEELSKYFKNH

SEQ ID NO: 9 - protein, 25 aa, Plasmodium falciparum
YEKAKNAYQKANQAVLKAKEASSYD

SEQ ID NO: 10 - protein, 27 aa, Plasmodium falciparum
AKEASSYDYILGWEFGGGVPEHKKEEN

SEQ ID NO: 11 - protein, 28 aa, Plasmodium falciparum
PEHKKEENMLSHLYVSSKDKENISKEND

SEQ ID NO: 12 - protein, 41 aa, Plasmodium falciparum
MLSHLYVSSKDKENISKENDDVLDEKEEEAEETEEEELEEK

SEQ ID NO: 13 - protein, 34 aa, Plasmodium falciparum
EEENDKKKEQEKEQSNENNDQKKDMEAQNLISKN

SEQ ID NO: 14 - protein, 53 aa, Plasmodium falciparum
NLISKNQNNNEKNVKEAAESIMKTLAGLIKGNNQIDSTLKDLVEELSKYFKNH

SEQ ID NO: 15 - protein, 371 aa, Plasmodium falciparum
MNKIYNITFLFILLNLYINENNFIRNELINEKNHNLRNGSMYNNDKILSKNEVDTNIESNENSIHESGHKIDGEEVLKANVDDITYKKKNVDDSEIPFSGYDIQATYQFPSTSGGNNVIPLPIKQSGENQYTVTSISGIQKGANGLTGATENITQVVQANSETNKNPTSHSNSTTTSLNNNILGWEFGGGAPQNGAAEDKKTEYLLEQIKIPSWDRNNIPDENEQVIEDPQEDNKDEDEDEETETENLETEDDNNEEIEENEEDDIDEESVEEKEEEEEKKEEEEKKEEKKEEKKPDNEITNEVKEEQKYSSPSDINAQNLISNKNKKNDETKKTAENIVKTLVGLFNEKNEIDSTINNLVQEMIHLFSNN

SEQ ID NO: 16 - protein, 211 aa, Plasmodium falciparum
SETNKNPTSHSNSTTTSLNNNILGWEFGGGAPQNGAAEDKKTEYLLEQIKIPSWDRNNIPDENEQVIEDPQEDNKDEDEDEETETENLETEDDNNEEIEENEEDDIDEESVEEKEEEEEKKEEEEKKEEKKEEKKPDNEITNEVKEEQKYSSPSDINAQNLISNKNKKNDETKKTAENIVKTLVGLFNEKNEIDSTINNLVQEMIHLFSNN

SEQ ID NO: 17 - protein, 21 aa, Plasmodium falciparum
SETNKNPTSHSNSTTTSLNNN

SEQ ID NO: 18 - protein, 27 aa, Plasmodium falciparum
LNNNILGWEFGGGAPQNGAAEDKKTEY

SEQ ID NO: 19 - protein, 33 aa, Plasmodium falciparum
PQNGAAEDKKTEYLLEQIKIPSWDRNNIPDENE

SEQ ID NO: 20 - protein, 53 aa, Plasmodium falciparum
LLEQIKIPSWDRNNIPDENEQVIEDPQEDNKDEDEDEETETENLETEDDNNEE

SEQ ID NO: 21 - protein, 42 aa, Plasmodium falciparum
EEEKKEEKKEEKKPDNEITNEVKEEQKYSSPSDINAQNLISN

SEQ ID NO: 22 - protein, 52 aa, Plasmodium falciparum
NLISNKNKKNDETKKTAENIVKTLVGLFNEKNEIDSTINNLVQEMIHLFSNN

SEQ ID NO: 23 - protein, 424 aa, Plasmodium falciparum
MKKIVNIIFYILYLYIYKRNLVQNENVNKSNLRKGLSTNNSENGIKSLKDEDEHINIIGDDFSAFSYGGYPIYETTGSLGTGVESVKAIDGESGTSMDSKPKENKISTEPGADQVSIGLVNESDSSLENDKKKKENVKKEMLGTEKEGSPDSHDSSKEKLNLNDNSKWSDFLKNIVTFGGFGPTVVHDVSDTLSDISKDEVTQKTTKDIGSTLLDFFLPLPTKNTNTYEKKNENKNVSNVDSKTKSNEKGRPPTYSPILDDGIEFSGGLYFNEKKSTEENKQKNVLESVNLTSWDKEDIVKENEDVKDEKDEDDEEEEEKYENEIIKQPEDILDEEEVLEEEILEENKNDTVDTSDLEKKNIPDLSNDNNYYSLIYKNYKDNDKSEKTAQTLITALISLLNGKNELDATIRRLKHRFMEFFTYN

SEQ ID NO: 24 - protein, 197 aa, Plasmodium falciparum
YEKKNENKNVSNVDSKTKSNEKGRPPTYSPILDDGIEFSGGLYFNEKKSTEENKQKNVLESVNLTSWDKEDIVKENEDVKDEKDEDDEEEEEKYENEIIKQPEDILDEEEVLEEEILEENKNDTVDTSDLEKKNIPDLSNDNNYYSLIYKNYKDNDKSEKTAQTLITALISLLNGKNELDATIRRLKHRFMEFFTYN

SEQ ID NO: 25 - protein, 24 aa, Plasmodium falciparum
YEKKNENKNVSNVDSKTKSNEKGR

SEQ ID NO: 26 - protein, 26 aa, Plasmodium falciparum
SNEKGRPPTYSPILDDGIEFSGGLYF

SEQ ID NO: 27 - protein, 29 aa, Plasmodium falciparum
GIEFSGGLYFNEKKSTEENKQKNVLESVN

SEQ ID NO: 28 - protein, 32 aa, Plasmodium falciparum
STEENKQKNVLESVNLTSWDKEDIVKENEDVK

SEQ ID NO: 29 - protein, 33 aa, Plasmodium falciparum
DTSDLEKKNIPDLSNDNNYYSLIYKNYKDNDKS

SEQ ID NO: 30 - protein, 52 aa, Plasmodium falciparum
SLIYKNYKDNDKSEKTAQTLITALISLLNGKNELDATIRRLKHRFMEFFTYN

SEQ ID NO: 31 - protein, 697 aa, Plasmodium falciparum
MKKIYSIFFSLFILNLHIYIKNIKCNDLINYNDSNLRNGLLNNSLDLTNGLNNKDNSFIDSKIEEHENKSYQNKDNNISIVGQDVPITSVYSSKIINANDLEGNSIDDTKGLSVTNSGFDDGSAFGGGLPFSGYSPLQGNHNKCPDENFCKGIKNVLSCPPKNSTGRNGDWISVAVKESSTTNKGVLVPPRRTKLCLRNINKVWHRIKDEKNFKEEFVKVALGESNALMKHYKEKNLNALTAIKYGFSDMGDIIKGTDLIDYQITKNINRALDKILRNETSNDKIKKRVDWWEANKSAFWDAFMCGYKVHIGNKPCPEHDNMDRIPQYLRWFREWGTYVCSEYKNKFEDVIKLCNIQQFTNQDDSQLLEISKKDKCKEALKHYEEWVNRRRPEWKGQCDKFEKEKSKYEDTKSITAEKYLKEICSECDCKYKDLDNTFKEFKDNVTLLKAVIDNKKNQDSLTTTSLSTSINSVRDSSNLDQRGNITTSQGNSHRATVVQQVDQTNRLDNVNSVTQRGNNNYNNNLERGLGSGALPGTNIITEEKYSLELIKLTSKDEEDIIKHNEDVREEIEEQQEDIEEDEEELENEGEETKEEDDEEKNETNDTEDTDDTEDTEDIEEENKEKELSNQQQSEKKSISKVDEDSYRILSVSYKDNNEVKNVAESIVKKLFSLFNDNNNLETIFKGLTEDMTDLFQK

SEQ ID NO: 32 - protein, 190 aa, Plasmodium falciparum
DNVNSVTQRGNNNYNNNLERGLGSGALPGTNIITEEKYSLELIKLTSKDEEDIIKHNEDVREEIEEQQEDIEEDEEELENEGEETKEEDDEEKNETNDTEDTDDTEDTEDIEEENKEKELSNQQQSEKKSISKVDEDSYRILSVSYKDNNEVKNVAESIVKKLFSLFNDNNNLETIFKGLTEDMTDLFQK

SEQ ID NO: 33 - protein, 25 aa, Plasmodium falciparum
DNVNSVTQRGNNNYNNNLERGLGSG

SEQ ID NO: 34 - protein, 27 aa, Plasmodium falciparum
LERGLGSGALPGTNIITEEKYSLELIK

SEQ ID NO: 35 - protein, 28 aa, Plasmodium falciparum
KYSLELIKLTSKDEEDIIKHNEDVREEI

SEQ ID NO: 36 - protein, 28 aa, Plasmodium falciparum
LTSKDEEDIIKHNEDVREEIEEQQEDIE

SEQ ID NO: 37 - protein, 34 aa, Plasmodium falciparum
EENKEKELSNQQQSEKKSISKVDEDSYRILSVSY

SEQ ID NO: 38 - protein, 51 aa, Plasmodium falciparum
RILSVSYKDNNEVKNVAESIVKKLFSLFNDNNNLETIFKGLTEDMTDLFQK

SEQ ID NO: 39 - protein, 405 aa, Plasmodium falciparum
MNKFLNIIFYIFLILNFSFFQSNATSKEIQKDEQKNLRNGSSINNNKNIENKNDNIETQYEASEYIEKQNDILNMYNDEKEKNNNNSLDTNVTKNTVIDNSNKFQSIEDNNVYNKGIFVGTGIKLNDSQTTSDNYKNERYQIDDEKLKYGGSFDTIFSGFVNLLTPSSPTQNDGSTGRNVPPPSEPNVDTPDPPTAPAPVKVPEDAKLSSSPRPEGPRANNRNENNQNTDPYNHYFAWEIGGGAPTYKPENNKNDNILLEHVKITSWDKEDIIKENEDTKREVQETEDTDETEDTDETEETEDMEDENEIVEDQLQENEDDEDNVNLEDINKNTRNDIFEEQIKLDSTQDDKAQKLISNEYKKTEEKKSLEDHVNLLFNFLQTNNQLDPSLKDLENELTFFLNNY

SEQ ID NO: 40 - protein, 192 aa, Plasmodium falciparum
PEGPRANNRNENNQNTDPYNHYFAWEIGGGAPTYKPENNKNDNILLEHVKITSWDKEDIIKENEDTKREVQETEDTDETEDTDETEETEDMEDENEIVEDQLQENEDDEDNVNLEDINKNTRNDIFEEQIKLDSTQDDKAQKLISNEYKKTEEKKSLEDHVNLLFNFLQTNNQLDPSLKDLENELTFFLNNY

SEQ ID NO: 41 - protein, 26 aa, Plasmodium falciparum
PEGPRANNRNENNQNTDPYNHYFAWE

SEQ ID NO: 42 - protein, 22 aa, Plasmodium falciparum
YNHYFAWEIGGGAPTYKPENNK

SEQ ID NO: 43 - protein, 27 aa, Plasmodium falciparum
PTYKPENNKNDNILLEHVKITSWDKED

SEQ ID NO: 44 - protein, 29 aa, Plasmodium falciparum
ILLEHVKITSWDKEDIIKENEDTKREVQE

SEQ ID NO: 45 - protein, 35 aa, Plasmodium falciparum
VNLEDINKNTRNDIFEEQIKLDSTQDDKAQKLISN

SEQ ID NO: 46 - protein, 52 aa, Plasmodium falciparum
QKLISNEYKKTEEKKSLEDHVNLLFNFLQTNNQLDPSLKDLENELTFFLNNY

SEQ ID NO: 47 - protein, 762 aa, Plasmodium falciparum
MIYILSIVFYIFFLHIDIYVNIYSTCFVVNEGNPNLRNNIINDDELKGKAYNNTIDANNQNIEYNKNLKHNVNSSHISKFSDIMDQEDKGDNENSHDIKFEEKKNINKSLDAESNYGINEISITGNDSNSDNSNQNIFPDGSELAGGIPRSIYTINLGFNKCPTEEICKDFSNLPQCRKNVHERNNWLGSSVKNFSSDNKGVLVPPRRQSLCLRITLQDFRTKKKKEGDFEKFIYSYASSEARKLRTIHNNNLEKAHQAIRYSFADIGNIIRGDDMMDTPTSKETITYLEKVLKIYNENNDKPKDAKKWWTENRHHVWEAMMCGYQSAQKDNQCTGYGNIDDIPQFLRWFREWGTYVCEESEKNMNTLKAVCFPKQPRTEANPALTVHENEMCSSTLKKYEEWYNKRKTEWTEQSIKYNNDKINYTDIKTLSPSEYLIEKCPECKCTKKNLQDVFELTFDGKALLEKLKKEESPVSNSVNALPEPGQITLPDPSLKQTTQQENQPVVETPVTTAVINEHQGQTEPNKGDNNNERENHESNVGSIQEVNQGSVSEESHSKTIDPSKIDDRLELSSGSSSLEQHSKEDVKKGCALELVPLSLSDIEQIANESEDVLEEIEEEINTDGEIEYITEEEIKEDIEEETEEDIEEETEEETEEETEEEADEETVKEIEDKPEQEIKNKSLEEKQIDKNTDTSEKKGFNNSEKDEKARNLISKNYKNYNELDKNVHTLVNSIISLLEEGNGSDSTLNSLSKDITNLFKN

SEQ ID NO: 48 - protein, 226 aa, Plasmodium falciparum
HESNVGSIQEVNQGSVSEESHSKTIDPSKIDDRLELSSGSSSLEQHSKEDVKKGCALELVPLSLSDIEQIANESEDVLEEIEEEINTDGEIEYITEEEIKEDIEEETEEDIEEETEEETEEETEEEADEETVKEIEDKPEQEIKNKSLEEKQIDKNTDTSEKKGFNNSEKDEKARNLISKNYKNYNELDKNVHTLVNSIISLLEEGNGSDSTLNSLSKDITNLFKN

SEQ ID NO: 49 - protein, 33 aa, Plasmodium falciparum
HESNVGSIQEVNQGSVSEESHSKTIDPSKIDDR

SEQ ID NO: 50 - protein, 29 aa, Plasmodium falciparum
SKTIDPSKIDDRLELSSGSSSLEQHSKED

SEQ ID NO: 51 - protein, 29 aa, Plasmodium falciparum
EQHSKEDVKKGCALELVPLSLSDIEQIAN

SEQ ID NO: 52 - protein, 33 aa, Plasmodium falciparum
ALELVPLSLSDIEQIANESEDVLEEIEEEINTD

SEQ ID NO: 53 - protein, 41 aa, Plasmodium falciparum
EIEDKPEQEIKNKSLEEKQIDKNTDTSEKKGFNNSEKDEKA

SEQ ID NO: 54 - protein, 61 aa, Plasmodium falciparum
NNSEKDEKARNLISKNYKNYNELDKNVHTLVNSIISLLEEGNGSDSTLNSLSKDITNLFKN

SEQ ID NO: 55 - protein, 272 aa, Plasmodium falciparum
MWIVKFLIVVHFFIICTINFDKLYISYSYNIVPENGRMLNMRILGEEKPNVDGVSTSNTPGGNESSSASPNLSDAAEKKDEKEASEQGEESHKKENSQESANGKDDVKEEKKTNEKKDDGKTDKVQEKVLEKSPKESQMVDDKKKTEAIPKKVVQPSSSNSGGHVGEEEDHNEGEGEHEEEEEHEEDDDDEDDDTYNKDDLEDEDLCKHNNGGCGDDKLCEYVGNRRVKCKCKEGYKLEGIECVELLSLASSSLNLIFNSFITIFVVILLIN

SEQ ID NO: 56 - protein, 9563 aa, Plasmodium falciparum
MKKESYRFLNISINNGSDKKKKSNFFVKIKNGTDLKDTKKDRIRFHFYFYFFIVKIILLSLLIWTVIYSNNCSNGKYKSTLYIVGNHLRFRGFRILAENEYEMKTKYKTLMVNIDDNDLGKRGNKIKPKHKKVEINLNDNNLSNNESKRKSRRKKVKVNLKDNLAKREGKMKRRNKKEKRRKEKDNKKMNELKLKREYKESYLLDNKSDMDVIRNDKFSYFTLYKNNLFPNSNNYFLHMLKTYDEENKGIDENTDINENVEENEYVDKNTEGDKDGDEDKGGGESEGGDGHGSAGDSAGGDRGGDENKDKDNEENKDKKGNKDDDDEEEEEEEEDDEEKEEKDEKDEKDEKDEKDEKDEKDEKDEKDEKDEKDEKDEKDEKGEKDESKGEEKFLKEEKMPKKEENMQDKIERDKEFEGFKDEYFTQMEGGAYGITVEHEGQKLRETLTEGVEGYEKVIEEMEQTKLDEFLLPTNEGKSDDFVSEMEEERLFNFVSYMEEEVKDKMFIEREQGTEEEVIHEDLSDEKIGIEKKELETFVQDVSDEVLQDEQLIEEEKLTEEEKLTEEEKLTEEEKLTEDEQLIEEEKLTEEEKLTEEEKLTEEEKLTEEEKLTEEEKLTEEEKLTEEEKLTEEEKLTEEEIFIEEDKISPKEVEEPLEDVLMEKMEKEYKEILHEGKSVVTQDMDEKLLSENLEDDLIPEEIIEELVDEELVEEVTAEEIVEEFVAEVEIEEKIPKELVEEVMPEEDVDEVVPEELVEEVVPEELIEGVIPEELVEDVIPEKVLEKVIPEEIIEELVLEEVVEEIKHEELVEEEIPEEVTEEVIPDEVVEEVIPEELIEKVVKEELVEKVVAEEIVEEVVPEELVEKVVAEEIVEEVIPEELIEEVITEKPAEEVIPEELVEEVIPKEIVEEVLPEEVVKEVIPEEVVEEVIPEELVEEVIPEEIVEEVVPEELVEEMKPEEVVEEVISEELVEEMKPEEVVEEMKPEEVVEEVTPEKVVEEVVPEELVEEMKPEEVVEEVISEELVEEMKPEEVVEEVTPEKVVEEVVPEELVEEMKPEEVVEEVISEELVEEMKPEEVVEEVISEELVEEMKPEEVVEEVTPEKVVEEVVPEELVEEMKPEEVVEEVISEELVEEMKPEEVVEEVTPEKVVEEVVPEELVEEMKPEEVVEEVISEELVEEMKPEEVVEEVVPEELVEEVIPEEVVEEIIPEEVVHEAKHEELFEKTVPEVEVQEIIPKELVEVIPEEVLPEELIEEVIPEEIIEEVIPEEVVEEVIPEEIVQEVIPEDLMEEVVPEEIIEEKILEEIVEEEIHEEIVEEIISEEVVEEVVPAEVVEEMIPEKLVEEVIPEELVEEVISEELVEEVVPVEVLEEVVPVEVLEEVIPEEVVEEVIPEEFIEEMIPEEIVEEVVPEVVEEVIPEELVEEVVPVELLEEVIPEELLEEVIPEELVEEVVPEELVEDVIPEELIAEVVSEELVEEEIPEEVLEEVIPEELVEEVIPEELVEEVIPEVLVEEVIPEELVEEVIPEVLVEEEVPEELVEEVIPELLVAEVIPEELVAEVIPEEFVEEVIPEEVVEELVPEELVEEVIPEEIVEEVVEEVVEEIIPEEVIEEVIPEEIVKEVVPEVLVEEVVPEEIVEEVVPEEIVEEVVPEELVEEVVPEELIEEVIPEELVEEVIPEVLVEEVIPEVLVEEMVLEELVEEVIPEVLVEEMVPEEVVEKMVLEEVVEEVIPEEVVEEVIPEEDVEQVIPEELIEEVVPEEVIEEVITEEVVEEVLPEELVEKVVEEEILEEVIPEELVEEVVREELIEEVVTEELVEKVVEEEIVEEVVLAEVVEEVIPQEIVEEVIPEEVVEEVIPKEIVEEVIPEELVEEVVPEELVAEVIPEELVAEVIPEELIEEVVTEELVEEVIPEEVVEEVIPEEVVEEVVPEELVEEVVPEELVEEVVPEEIVEELLPKEVVEEVIYEEQVEEVIPEELVAEVIPEKLVEEVIPEELVEEVIPEELVEEVVPEVVEEVVPEELVEEVIPEELVEEVIPEVLVEEEVPEELVEEVIPEELVEEMLPEELIEVVVPEELVEEVVPEELVEEVVPEEVVEEVIPEELIEELVPEVEIEEILPEELIEELVPEEIIEEVIPKELIEEVIPEVVVEEVVPEVVEEVVPEIVEEVVPEVVEEVVPEEIIEEKISEEVVEEVLPKEIVEEVIPEELVEEVVPEELVAEVIPEELVEEVIPEVLFEEEIPEVVVEEVVPEVVEEEIPEVVVEEVVPEVVEEVIPEELVEEVIPEELIEEVIPEEVAEEVLPEELIEEVIPEELVEEVVPEELVAEVIPEEIVEEVVREELVEEVVPEEVVEEVIPKEIVEEVVSEEVVEEVIPKEIVEEEVPEELVEVVPEELVEEVVPEELVEEVVPEELVEEVVPEELVEEVVPEELVEEVVPEVVEEVQEQLVEEFIPEEVVEELVPEELVEEVIPEELVEEVIPEEIVEEVLPEEVVKEVIPEEVVEEVIPEELVEEVIPEEIVEEVLPEEVVKEVIPEEVVEEVIPEELVEEVIPEELVEEVIPEELVEEVVSEELVEEVIPEEIVEEVIPEELLEEVVEEVVPEIVEEVVPEVVEEVITEEVIPEELIKEVIPEELVEEVIPEEIVEEVIPEEIVEEVISEEVVEEVVPEVVVEEVIPEEIVEEVLPKEIVEEVISEKVVEEMIPEELVEEVIPEEVVEEVIPEVEIEEILPEELIEELVAEEVIEEVIPKELIEEVIPEKLIEDVVPEEIVEEVLPEEVVKEVIPEEVVEEVLPEELVEEVIPEVVEEVVPEELVEEVLPKEVVEEVIPEVEIEEILPEEIIEELVAKEVIEEVIPKELIEEAITEEVVEEMIPEEIIEEVVPEEVIEEVITEEVVEEVVPEEVIEEVITEEVVEEAIPEEVVEEVIPEVEIEEVLPEELIEELVPEEVTEEVITEEVVEEAISEVVEEVIPEEIVKEVIPEEVVEEIITEEIAEEIIPKELVEEVIPEEVVVEIIPEKLVEEFVSEELVEELVPEEIVEKVVPEELVEEIVPEELVEEVVPEELVEEVIPEELVEEFIPEEVVEEVLPEQLVEEVISEVVEEVVPEELVEEVIPEEVVEELVAEEVIEEVIPKELIEEAITEEVEEVIPEEIVEEVIPEEVVKEVIPEVEIEEILPEELIEELVAKEVIEEVITEEVAEEVIPEEIVQEVIPEEVVEEIITEVEIEEVLPEELIDEVVPEEVTEEVITEEVMPEEVVKEVIPEEIAEEVIPKELVEEVIPEEVVEEIIPEVEIEEVLPEEVIEEVVPEVEIEELIPDEVVEEVLPEELVEEVIPEEVAVEVVPEEVIEEAVPEEIVEEFIPEEQIEEVIQEEIIEQVVPEELIEEVVPEEIIEEVIPEEIVEEVIYEEVIPEELVEEVIAEKLVKEIVPEQVREEVTLEEIVEEMIPEEFVEEVAPEVEIEEIIPEELIEEVIPEVLVEEAVPEELIEKVIPEVLVEEIIYKEGIPEVLIEEVIPEELVQEVIPEEIVEEVVPEEFIEEMIPQEVVKEVITEKFIEEMIPEEVVEEVIPEEFIEEMIPEVVVEEVVPEELVEEMLPEELIEVVVPEELIEEVIPEELVEEVVAEELVEEVIPEELVEKVVPEVVEEFIHEVVEEVVPEVVEEVVPEVVEEVVPEVVEEVVPEVVEEVVPEVVEEVVPEVVEEVVPEVVEEVVPEVVEEVVPEVVEEVVPEELVEEVIPEVLFEEEIPEELVEVVPVELLEEAIPEELVEEVIPEELVEEVIPEELVEEVIPEELVEEVILEELVEEVIPEELVEEVIPEELVEEVIPEVLVEEEIPEKLVEEDIPEKLVEEVVPEELVEVVIPEELVEEVIPEELVKEVIPEELVKEVVPEELVEEEIPKVVEEVLPEELVEEVMLEEVVEEVVPEIVEEVVPEELVEEVVPEVVEEVVPEEIVEEVIPEELVEEVVKEELVEEVVKEELVEEVVKEELVEEVIPEVLVEEVVPEELLEEVIPKVLVEEVIPELLVEEVVPEVIEEVVPEVVEEVVPEELLEEVIPEVLVEEEIPEKLVEEVVPEELVEEVIPEVLVEEVVPEELVEEVISEELVEEVIPEELVEEVIPEEVVEEVVPEVVEEVVPEVVEEVVPEVVEEVVPEVVEEVVPEVVEEVVPEVVEEVVPEVVEEVVPEVVEEVVPEVVEEVVPEELIEEVIPEEIVEEVIPEELVAEVIPEKLVEEVIPEELVEEVIPEELVEEVIPEELVEEVLPEEVVEEAVPEVVEEIVPEELIEEVIPEELIKEVVPEEVIEEVITEEVVEEVLPEEIVEEVLPEEVIEEVVPEELVEEVLPEEVVEEVVPEELVEEVVPEELVEEVIPEELVEEVLPEEVVEEVVPKELVEELIPEELVEEVIPEELVEEVVPEELVAEVIPEELVEEVIPEELVEEVIPEELVEEEIPEELVEEVILEELVEEVVPEELIEEVVPEELIEEVVPEELIEEVVEKVIPEEIIEEVVPEEVIEEVITEEVVEEVVPEKVIEEVITEEVVEEVVPEEVIDEVITEEVVEEVVPEEVIEEVIIEEVVEEVVPEEVIEEVITEEVVEEAIPEELVEEVIPEVLVEEEIPEELVEEVILEELVEEVVAEELIEEVVEEVIPEKLVEEVIPEEIVEEVIPEELVEVVVPEELVEEVIPEELVEEVIHEELVEEVIPEELVEEVIHEEIVEEVIPEEVVEEVIPEEIVEEVVPEELLEEVIPELLVEEVVPEVVEEVVPVELLEEVVEEVITEEVIPEELIKEVISEELVEELIPEEVVQEVITEEVLEEVIPEEIVEELIPEKLIGEVVPEKVVEEVVLEEVVEEVIPEEIVEEVITEEVLAEEIVEEFVPEELVEEMLPEEVVEERVREVEIEEMVPEVLVEEVLPEVVEEVITEEVVEEMVPEEVVEEMVPKEIVEEVLPEEVVEEVIPEEVVEEMVPEVLVEEVVPEEIVEKVVPEEVVEEVVAEEIIEEVITEEVVEEIVPGEVVEEMVPEEIIEEVVPEEVIEEVITEEVVEEVIPEELVEEVIPEISVEVEIPEVLVEEVIPEKLVKVVPEELVEEVIPEELVEEVITEALVEEVVDVVVPEEIFEEVLPEEVVEEVIPEEVVEEMVPEEVVEEVVPEELVEEVIPEEVVEKVVPEQLVEKVVPEELVEKVLPEELVEEVVPEELIEEVVTEEVIEEIIPEEIIEEIIPEEVVEERVSIEVVEELVPEELIEEVVAEEIFEEVVPEKLIEEVVAEELIEEMVPEVVEEVVEEIIPEEVIEEVIPEEIREEIIPEEVVEEVIEEVIPEELIEEEISREIVEEVIPEEVVEEMMPEEVIEEVIPEEIREEMIPEEVVEEMIPEIEIEQVLPEELIEELVPEVEIEEILPEELIEELVPEGVIEEVIPKELIEEVIPEELIKEVVPEEVVEEVIPKEIVEEVVPEELIEEVIPEELIEEVVPEEMIEEVIPEELIEEVVPEEMIEEVIPEELIEEVVPEEVKEEVIPVELIEEVVPEEMIEEVISEEVVEEVIPEELVEEVLPEVFVEEIVPKELVEEVIPEEIVEEVIPEELVEEVIPEELVEEVISEELLEEVIPELLVEEVVPEVIEEVVPEVVEEVIPEVVEEVVTEELVEEVIPEEVVEEMIPGVEIEEVLPEELVEEVIPEEIVEEVISEEDFEEVIPEALVEEVIPELLVEEVVLEELIEEVIPEVVEEVIPEEVVEEVIPEEVVEKVVPEELVEEVIPEELVEEVIPEEVPEEVVPEELVEEVISEELVEEVIPEEIVEEVIPEEIVEEVMPEEVAEEVVPEELVEEEVPEELVEEVIPEVLVEEVIPEEIVEEVVPEEVVEVVIPEEFIEEIIPEEVVVEVTPEELIEEMKPEELFEEVIPKELIEEIIPEELIKEVIPEEIIEEVISKEIVEEVVEEEIIEEVIPEEIVEEVVPEELVEKKVPEEIVEEVIYEEFLEEIMPEELIEEMKPEELIEEIIPREIVEEIITEEVVEEMKPEELVEEMVPEEVVEEMVPEEVVEEMVPEEVVEEVITEKLIEEVVPEEIIEELIPEELVEEVIPEKLIEEMIPEEVVEEMLLEEVVEEVVPEVEIEEMIPEQLVEEVVPEELVEKEIPEVVEEIITEEVVEEMVPEEVVEEMVPEEVVEEVILEKLIEEVVPVEVIEEVVPEEVIEEVIPEKLIEEIIPEVLVEEVVPEELIEEVIPEVLFEEVVPEVVEEVVPEELVEKVVPEEIVEEVIPEFVEEVISEEIVEEVVTEELIEEMIPEEVVEEVIPEELVEEVVPVELIEEVVPVELLEEVIPEELVEEVVPVELIEEVVPVELLEEVIPEEVVEEVIPEVVKEVVPEVVEEVVPEVVEEVVPEVVEEVVPEVVEEVVPEELIEEVIPEELIKEVLPEEVIEELKPEELIEEIIPEEVVEEVIPEELIEEMIPELLVEEEVPEELVEEVIPEVLVEEMVPEEIVEEVIPEELIAEFAPEELFEKVIPEEVVEELVSEELVEEVLPEVVEEVLPEVFEEVIPEEVIEEIVPEEVMEEVVPKELIEEVIPEELIEEVIPEEVAEEVVPEKLIEEVIPEELIKEVVPEELIEEVITEEVVEEAISEELVEEVVPEEVVEEVIPEELIEEVVPEELIEEIIPEELVEEVIPEELVEEVVPEELVEEVIPEELVEEVVPEELVEKLIPEELVEEVIPELLVEEVVPEEVVEELIPEELVEEVIPEELVEEVIPEEVPEEVIREELVEEVIPEELVEEVIPEEVPEEVVPEELVQEVIPEELVEEVVHEEVPEEVVPEKLVEEVIPEELFEEVVPEEVPEEVVPEELVEEVISEELVEEVIPEELVEEFIPEELVEEVIPEELVEEVIPEELVEEFIPEELVEEVIPEELVEEVIPEVLVEEEIPEKLVEEVVPEELVEEVIPEVLVEEVVTEEVPEEVVPEELVAEVVPEELVKEVIPEELVEEVIPEEIVEEVIPEEVVEEVVPEELVEEVIPEEVVEEVIPEELVEEVVPVELVEEVVPEELVEEVIPEELVEEVIPEEIVEEVIPEEVVEEVIPEEIVEEVISEELIEEVVPVELLEEVVPVEVLEDVIPEEVVEEVIPEEFIEEMIPEEIIEEAIPEEIVEEVIPEVVEEVVPEELVEEVIPEEVVEKVVPEELVEEVIPEELVEEVIPEEVPEEVVPEELVEEVISEELVEEIIPEELVEEVIPEEVVEEVVPEELVEEVIPEELVEEVIPEELVEEVIPEVVEEVIPEKLVEEVVPEELIEEMIPEEIVEEVVPEVVEEVIPEELIEEVIPEELVEEVIPEKLIEEMIPEELVEEVILEEVVEEVIPEEVVEEVLPEELVEEVVPEELVEEVAPVELLEEVIPEELLEEVIPEELVEEVIPEELVEDVIPEELVEEVIPEELVEEIIPEELVEEVIPEVLVEEEVPEELVEEVIPEELVEEVIPEELVEELIPEVLEEVIPEKLVEEVVPVELLEEVIPEELIEEVVPEVLVEVIPEKVVEEVIHEEIVKEVVPEELVEEVVPEEIVEEVVPEEVLEEVIPKVLLEEEIPEKLVEEVIPEELIEEVVPEELVEEVMPEEVVEEVVPEELVEEVIPEEVVEEVIPEELVEEVVPVELLEEIVPVELLEEVIPEELVEEVIPEELVEEVVPEELVAEVIPEKLVEEVIPEKLVEEVIPEELVEEVVPEELVAEVIPEKLVEEVIPEELVEEIIPEELVEEVVPEELVEEVVPEELVEEVIPEELVEEVIPEVLVEEEVPEELVEEVIPEELVEEMLPEELIEVVVPEELVEEVVPEELVEEVVPEEVVEEVIPEELIEELVPEVEIEEILPEELIEELVPEEIIEEVIPKELIEEVIPEVVVEEVVPEVLVEEVVPEELVEEVIPEVLVEEEVPEELVEDVIPEELVEEVVPEELVEEVIPEEVVEEVLPEELVEEVVPEEIVEEVIPEELVEEEVPEELVEEVIPEEVVEEVIPEEVPEKVIPEKLVEELIPEEVVEELIPEEVVEEMVPIEVVEEVVPTEVLEEVIPEIVVEEVVPEELVEEVIPEELVEEVIPEIVVEEVVPEELVEEVIPEELVEEVVPEELVEEVVPEEIVEELLPKEIVEEVIYEEQVEEVIHEELVAEVIPEEVVEEVVPEVVEEVVPEIVAEVIPEEVVEEVVPEVVEEVVPEVVEEVIPEEVVEEVIPEEFIEEMIPEEIVEEVVPEVVEEVIPEELVAEVIPEELVEEVIPEVLFEEEIPEVVVEEVVPEVVEEEIPEVVVEEVVPEVVEEVIPEEVVEELIPEEVVEEMVPIEIVEEVVPTEVLEEVIPEIVVEEVVPEELVEEVIPEELVEEVVPEELVEEVVPEVVEEVVPEVVEEVVPEELVEEVIPEVVVEEVVPEELVEEVIPEELVEEIIPEEIVEEVIPEELIEEVVPEVLVEEVIPEELVEEVIPEELFEEVVPEELVAEVIPEEIVEEVIPEELIEEFVPEELVEEEVPEELVEEVIPEVLVEEVIPEEFVEEVIPEEIVEEVIPEEIVEEVIPEEVVEEVVPEIVAEVIPEEVVEEVVPEVVEEVVPEVIEEVVPEVIEEVVPEVVEEVVPEVVEEVVPEVVEEVVPVEVLEEVIPEEVVEEVIPEEFIEEMIPEEIVEEVVPEVVEDVIPEELIAEVVSEELFEEEIPEELVEVVPVELLEEVIPEELVEEVIPEELVEEVVPEELVEEVVPEELVEEVIPEELFEEVVPEELVEEVIPEEIVEEVIPEELIEEFVPEELVEEEVPEELVEEVIPEVLVEEVIPEEFVEEVIPEELVEEVIPEELFEEVVPEELVEEVIPEEIVEEVIPEELIEEVVPEVLVEEVIPEELVEEVIPEELFEEVVPEELVAEVIPEEIVEEVIPEELIEEFVPEELVEEEVPEELVEEVIPEVLVEEEVPEELVEEVIPEELVEEMLPEELIEVVVPEELVEEVVPEIVEEVVPEELVEEVIPEEVVEEVLPEKLVEEVVPEIVEEVAPEVVEEVIPEELVEEIIPEILVEEVVPIEVVEEAVPEVVVEEVVPEKIVEEVVPEKVLEEVIPELLVEEIVPIEVVGEIVPEEVVEKIVPMEVVEELLPEVVEEVPHEIVEEEVVKEVIPEDEKKVEIVEIIIEEKVEKIPKKKVIEKKKEKEKIRKPKKKVEKEIKPKEVKGVKGKLKKDVKAKHLKGSKVKITEDIQKKMEDDIKEKIMEKELKEEIKDKEYLRKVIPKEEKKEPIPKKGKSVEPKKEKQAGVKKEKVPETKKEKAPAPKKEKVQAPKKEKVPAPKKEKPAVPKKEKVPEPKKEKVPEPKKEKAPAPKKEKVQAPKKEKAPAPKKEKAPAPKKEKAPAPKKEKAPAPKKEKPAVPKKEKPAVPKKEKVPETKKEKVPETKKEKVPETKKEKVPVPKKEKVPAPKKEKVPAPKKEKVPAPKKEKPAVPKKEKVPETKKEKAPEPKKEKAPEPKKEKAPEPKKEKAPEPKKEKAPAPKKEKVPVPKKEKVPAPKKEKVPAPKKEKPAVPKKEKVPETKKEKEKDSQPKKEKAKETSRPPKKEKEKGK

SEQ ID NO: 57 - protein, 133 aa, Plasmodium falciparum
IPEEQIEEVIQEEIIEQVVPEELIEEVVPEEIIEEVIPEEIVEEVIYEEVIPEELVEEVIAEKLVKEIVPEQVREEVTLEEIVEEMIPEEFVEEVAPEVEIEEIIPEELIEEVIPEVLVEEAVPEELIEKVIP

SEQ ID NO: 58 - protein, 6093 aa, Plasmodium falciparum
MSNINNKDSSTEWNCKEDVGCVPPRRQNLNMERLDNENEDSVPDFMKKTFYLAAAGEGKKLREKHDESCDEFCDAWNRSLADYKDIFQGKDMWNDGKYGEAKNHIKNAFGDMNNRKTMLNEIEKGIKDETFSRENGLDVCKSQCEERSRDDTEDQFLRFFAEWEEEFCDGLNKHEEQLKSCTKDINCDIKCSNFKDWLETKKDEYDIQSRVFEKKYANDNKSKHLNYLKEGMNKCKVKNPEMVFKSGFANVAECRNLNVEGAGNKNSNNLKDLDSNSDKDGIVSESYKATKKNGESIMDRIPKSFNKLFGYFSGSQEEEQKENDVSHRNNYDNILVDKFHRSSLLDKLDDRMFFDELNRDNIMEEVLSKIPEPIIREAPKYVPKKPVPPQHIPRGDNVPRNIDVNGSKDEYSPETESANSKIKPTYEENDEDKSKISIETSEIDRDKEPFRISEEKKVVKEDVQELENIEYEFDETFDFFDEDAKRNIDDIRKDIQSQIMKSVENYNSEKEEFKRNIETQLIESGDGMNAGNYSSALQDNSTEIPTMVLVPGVLTVFLLTIIWVLVYKHSLIDRVHGTGKTKKEEKMKELESEEFPKEKYNIEDMEETEKENEIEKIMDENKETEQTEEGNTEEFVQEKELNQETLENEIIVDHIKEEEDTRNVKEQESVLEESPIEELPVENNIGKINEEVEEFILNEIPLEEQVPKELPQEEIEEIVVEELPIDEHLSSEETTVTEEDTFKGQLINEEKPVEEKSVSEEIPVEEKSVSEEIPVEEKSVSEEIPVEEKSVSEEIPVEEKNVSEEIPVEEKNVSEEIPVEEKNVSEEIPVEEENVSEEIPEGGIAIEDVPVDEETVTEEITVDEKIYDKLPNEIETVNEEMPVEDETLTEQISSEHERVPEEIIEEKPFTEGEETESLTDEIVEEGVVTDDIPEEQIITEKVQEEEEFVTGELSEEDIINEKVQEEDESVTEELPEEDIINEKVQEEEESAYQEIVQDGSVTKDVEYKELVNDDVRDKENFVIEEDPFKGQLINEGLPVEEEFVTKELPVKEESVFEELTEEDQSVTKEIPVEEHSVFKEVDEIESVTDEIVEEEGSVNEEVEEEVSVSGEVDETEYVTEEVEETELVNEEVLKEEGSASEKVVKEEGSASEKIVEEEGSVTEETASEEIVEEEGSVTEESSSEEIVEDEGSVTEESSSEEIVEEEGSVIEESASEVIVEDEVSASKEIVEDEASVTEEVVEEEGAVSDEVQVTESVEDEIINQGIVDEVIVEQEASVTDEIVKEDESVIEEIAVEETVTEVVEETKPMDEEIVDQGSVVENVEEKKTMDEEIVDQGSVVENVEEKKTMDEEIGDQGSVAEKVEEEELVTEEVIEREGSINEDIVKEASITEEVEQIEPVTGKVEKIESITDEIKEQLVPEDIKEEQLDFEEIVAQRASVNDEKVEVASITEEVEEEEKSVSEEVLEEEGSTTEKVVKGSSTEVVVEEQGSVTENLLEEESASQGIVEKEEFVDEEDSVKDQNVFEKEGSVTEQLVEEEKGLINEDNEKEELITEMSEEIKSVNEEIEETDLSTEEIIKQQGLATYEFVEEEKSLTDKLLEEESVTKEVGETELSTQEVVDEKVSVTEEVIEEEKSVSEEVLEEGSATEEVVEEGSCTEVVVEEGSCTEVVVEEGSCTEIVVEKGSDTEIVVEEGSATEIVVEEGSATEVVVEEGSATEEVVEEGSVSEEMLEEEGSATEEVVEEGLSSDNVQKSKGVIENVGEIYSVKTAKDESMNEKIPLEKSSFVDDESFKGQGPTDNVSVEDVNSEDIINEHTPLEETKIEELPTEYITTADIHTKGETETKYNLIYEKINEEVEKAKFQEEKITENIPVERESVTEDIVQEPSLAQEVEQKESDTNEIEETKLANEKIIPEVSVTENVVEKEGLDTEEVLEEDESITEEIVEEEVSSSEEIVEEEESSSEEIVEEEESSSEEIVEEEESSSEEIVEEEESSSEEIVEEEESSSEEIIEEVSSTEEVLEEEGSVTEEIVEEEVSTTEEVKDIGSVSEEVLEEEGFGTEEFVGQQGSVIEEIVETESSTEKVLEDVGSNVEEIVQEEGPVAQEIVHEEVSTTEKHDEVDRSTTEEIVEKVGSVSEEIIVEEVSASEEIVEEGSVTEEVVEEEKLINEVGETESVTEEIVQKEVSDAEEVLGQEGSMNEEILEKESIVEEIVGPEGSVTEEIVDHGSFAEEVKEEELVTEEAVQYEGSVTEEIKEEESITENEAIEESAFAEIIEEKGPNTDEIVKEEGLDTEEIVNEVSVTDEVIEEEKLVNEQIVGEERSVTEKPVEVERSATEDLVEEEASVTEKVSVHEGSTTEQILDESVAEEIVEEEVSVDDKIIEEEVSVDEVVEEEGSVIEEIVEEEESVPEEILEEELSGSEEVLEDEWVTDAFMGQEGSVIEEIEEIVDGEGSITEEIVEDGSANEKIVEEEPSRVEEVLGKEGFVIEEIIEEGSVIEQVEDTKTVSEKSEESSAIEEVKEVKEEESISEKIVEKEESVTEEIVRQEESTTEKIVKDVSPTEDFVEQTDSVTEKVIEQEGSNTEVAEDVEEKESASDEHEQEDVSVNAQVTYEKKSVTKEIVDEVSRTEEIVEENGSVTEGVDETGSVTEEIIEEATVTEEVVEDGSVTEEVVEDGSVIQEVVEDGSVTEEIVQENGSVTEEIVEEEGSVNEEVEEEVSVSGEVDETEYVTEEVEEEGSVVEEIVEEEGSVSGEVDETEYVTEEVEEEGSVVEEIVEEEGSVSGEVDETEYVTEEVEEEGSVVEEIVEEEGSVSGEVDETEYVTEEVEEEGSVVEEIVEEEGSVVEEIVEEEGSVSEVVDETELVNDEIVEQAPFTEEVEEQVSVNDEIIEDASVAEAVEESESITESVSQEEETEKGFVIEKVEETGAVTEEIVQDGLITEEILEESESVNGEIINKESDAEEILETEFLTEEVVGQAGSTSEEIVEEEGSVTKEVEEKESVTEELVDEGSVTEELVDEGSVTEEVVEQGGSIAQEIVEEESATEEIIRDETNVEEVLEKEGSATEEIVQDGSGTNDFVGKQGSVIEEVVEEEISTTEEKLKEEASAIEEFVEEESIREDVLEESLVTENVVGQQESVTEEIVDGEGSFTEDIVEEEESVTEEIVVDEESVTKEIVEDEELVTEEIVEDEGSFTEEIVEDEGSFTEEVIEERSLIEEVEDTETVAEKEEGSVIKEIIDEKSLTEKIVEEEKSVTEEVEEKESVKEEVEEQRLVVEEEGSATEGIVEDRLATEGIVDDILVTEEIVEDGLATDEFVEQQGSIIEEVLDDEGSVTEEIVEEEGSPNEEIVEGVSVIEEDDNIEPVSEEIVEGSVTEEMIKEGLENEVILDEDSITEEALEKEGSVSEEIVEEMGSLTEEIVDEERSTSEDMIEEGSASEEIIQEESQVEEVVEEVSVIDEIVEEDELDTKEVVEEIEFNTEEVVEHKEEEGSVAEEIVQEEKEGSVNEEIIEEVGSITEEMVEQDVSDNEEIVEERSVIEEAEENVWIEKEVEEEGLDNEEVIDEEDSVSEQAEEEVYINEEILKESSDVEDVKVENELMNEEVNEETQSVAENNEEDKELDNYVVEETESVTEEVVVDEVPNSKEVQEIESIIEEIVEDGLTTDDLVGQQGSVIEEVVEEVGSDSEEIVEEASITEEVEKKESVTEDILVEESVTGDILVEGSVTEEVVGEEKLVSEEIVTEEGSVAQEIVEEDAPATEEIDEIESVTEEVVEEEGPVDEEIVQEEGSVTEEIIQGESKVEEVVEEQGSENEEIFVEEVSASQEIVQNESGTEEILEKVSASQEIVQDGSVTEQIIEEQKPVTEEVVNEEESITHEIIQEESHVEKVVQQGSVAEEVVENPVSVTEEIVEKEGSVTEDIGQEGYVAEEIVEEEEFDNEEILEEESVAEEFVEEGFDNEEIFVEQISDSEIVKEENSVNEEVLEEEGSYTEEILEEEGSYTEEILEEEGSFTEEILEEEGSYNEEILEEEGSYNEEILEEEGSYNEEILEEEGSYNEEILEEEGSATDYFVGQGSDNEEIIEEGSATDYFVGQGSDNEEIIEEGSATDYFVGQGSIIEEVLEEEGLDTEKVFENEGSATEFEETESFTEVVEETESVNENILEETSINEVQKIESITEDIKEQLVPEEIKEEQLDSEEIKEEQLDSEEIKEEQLVPEEIKEEQLDSEEIKEEQLDSEEIKEEQLDSEEIKEEQLDSEEIKEEQLVPEEIKEEQLDSEEIKEEQLVPEEIKEEQLDSEEIKEEQLDSEEIKEEQLDSEEIKEEQLDSEEIKEQKGSVNEEVVEEEGSVTEEIKEQEESVNEEVLEEVEETESIKEEIVEGGIATQEIIEEESDTKEVVEEEVIDSEKLVDAGSVTGEVMPEEVSVTDEVVEEGSTTEEVLEEQKSVNEEVVEDGLTIDDFVGLQGSTTEEVVEEDGSAIEKILEEETATEEIVEKQVSVTEDIVEKEGSVNEEIIEEASVAEEIIQGGSFTEEIVGQEESATEEVIDEEGLISNEIEEEEEKSVTEEMIEEVEEVSVDDEVEEVSVAEEIVEEELVDDEILPEELSATEDVIEEVRSVTDEIVQEESVCEEILEQEVSASEEYVDDKSVTDDFVGHERSVIQDVENTESVTEEIAEVDKSVIEEAVEKQGSVTEEKVQEGVSAIEEIEELESVTEEIAEEDKSVIEEAVEKQGSVTEEIVEEEELDTEEVLEDKSVTGDVVEQEGSGKDESEAKESFTEEVDELKSVKEEDQETEYISREIEEESATEQHSEQELSINKEVVETESLTKDIEEEKSTTQEILEETQSVNEEIVEEERDTDEVLKEKVSPSEEVIEEQASTTEEFVEERSSTDEIVEVEDLFTEEVKEREGSVTEEIVEEGSDTGEIVEEEGSDTEEILEEGSFNEEIVEEEGSITEEILQGSVTEEILQGSVTEEFVGQQGSVIEEIVETESAIEERVEEESATEEVDERESVTEVVEEEVSSSDEVVEGSIEEVIENEGSVTEEILEHEVSADENFVGQAVSVIEEVEGTESVTEEVVEETESVSEEIVEVSPTENVVQQTDSVIEEVVEQKEGSFNEEIDIRELGDDGVEEREKISTEEVVGQDKSATGDVEEVSSTEDEEEVSSTEGLEEVSSTEGLEEVSNTEDVEEVSSTEDVEEGSVAENVKETKSITEEVSVEEDIITDKVSVEQEVMAEASVEENILTEVPVEEEIMTEKLSVEDKALNEKIMSEEEIVIEDGNVHEVVPAEVSVTEEIPGVEETTNNESHVKGENVVNEVVVDDNSVNDEIQFDDDSSIEIYTVDSKDVFHKEENYDSFREEVRSDENIHIFRKKNENFVKKIENEKSSVGHVPTEYTSKENIAEEVPSHIMFKENVTEEVPKEVKYEENTVEEVFEEVTSKENIIEEAPGDINSEENIIEEVPEVVTSEEIVVQNDVNNINTNIDHMFDFDLDDILKIPEAQRKLNKLRTLVDVHLDVIEKMQRDEWKKNKRDFLYICLKEINKLSEDTLMKFYGSDSNKSANDNDTVMVIKILKDKWGTGRIVDTIANSLNKSYNSLYHNLYIEMEKDLLINKTETFNKWSKQHWNKLDNWKEEKWFKLFKRDLKIDMRNTYESDQNDEENNEESMNELSDELIKNNTSDNMRNEQKTLEKNKEYSNLSKDLGLIEKQKIIWKSWIVKNVNNIENWFDEMWFKNVVNELKEKNDVSNVLQENASEASVENYISDVEDSKDMTNSINDSEKSKIVASSSKTTNEEYIILSRKDLIYNIIVMVHMMVLDQFKYDELKYAKKRFLNRSIDKFIKEKKIKDKETVLDYYIDDIIKRIVEDTSHVNNIKEKAIDHYTSHDWFRLLRQGNKAQNSISQEVDILTEKYKKLISEEDNKKENNNNNDDEVKPELKDNIKCEENVSFNILRRSNKKDQLPLEEKKNKNGDLNNTLTESDGKKININEAIEESKNGNEDKNSGNMEKSRKPRDRRTERKEKDQDLRVQLLQDYENIFEQIQNMENQNKDKNKKETKNILKTSIDLDKNLLREYKKEKNIINQSEKEFSVNEN

SEQ ID NO: 59 - protein, 994 aa, Plasmodium falciparum
MKFFIPYVYIICVIFIINVIRTRGEEDDDNNNISGKSILGTSHNNISNIDLSSIPNLDSNIHASFSSDTKEWSPNNLTSKKKKKKKEIRPKDIMSNSDSSNTSSINKQNNNQIKSVLLKENKGVKITGPCNVNLSIFLVPHIYIDVETKYNNIELKYELDEFSDSIKFKDTTTELRTSDDTLMNTNFNVGVSRDTLDKDRLYNICAENKTFKFVVYIKDNILTLKWKVYETGVTNNKVDIRQYKMKELTRPITTIQIHSVSENKDTHLLESKNYVIKTDIPETCDVMATNCFLSGNINIEKCLECTLLVQNNDTSSECFTYVSNDVRENFNQIKAEAEDDENFRNYHLTDTINNILKRIYKINKNEGKKELITLEELDNFLKESITDYCKILREIDTNGTLVNHELGNNVDVFNNLIRLLKLHKNESISTLHNKLRNSAICMKYPDKWIEKKTGLILPNVVNNNIIYNNKYEKLNEEKKRKIYDNKDDSKISDIINIKKYIFTNNTLKYFNNDKQFCNSSFCNRLKDENNCISKIQIEDQGNCAISWIFASKYYLETLKCMKGYEPHAISALYIANCSKRKHKNRCNVGSNPLEFLQIIEENQFLPMDTNYLYSYTKVGNDCPDEEKNWVNLLKHTRMLNYNNKHRSTLSTKAYRAYESEHFKDKMDTFIKLIKDEIMNNGSVIAYVKAENVLGYELNGKNVQNLCGDKTPDHAVNIVGYGNYINDEDEKKSYWIVRNSWGKYWGDEGYFKVDMYGPSTCEDNFIHTVVVFNINMPKSKKSPVKITFPLYNYYLKYSPDFYHNLYYKNFNSKKSMKLVNASDEHKNIYSQEDKVNHKKGSKILNSEVTTSLLSQEISQRRGEDDDIDTLIGDSPDINEQEKNIKDEFNKSSITHNSVSSSNITKSNKNTNKVKIYHIIKHVKNTKIKIGFVKYDNYNTIGTNHTCSRSYSEDQEKHEGCIKFCELHWNECKDKTSPGYCLTKLKGSNECFFCYV

SEQ ID NO: 60 - protein, 1105 aa, Plasmodium falciparum
MKFHISFFLILYIVFFKNTIKSETTTDESATGSLSSDGSRVTTQARIEKPKQQPTLPTLAQETQPQQQQQQKEVGSGIGAEQKVESARPGAEVSQSDVERAGRSSGTGGSVGTKISPGSQGQGKVAGPQLPRLPQLPQSFEQSRNQQSSPVTPKRNGISPTNAKSPESVLPPAQSFTNLNKSTIPHTIPIKSSFLKYYKGVKITGSCGVQFQLVIVPHLFIYVETKENNIQLEPRFMKLNERIDFEKDKSNLKNKCDVNKKQSFKFILYLQHDLITIKWKVYEEKPDTTTRIAPGQVDLNVDVKRYKLPKLDQPVISIQIHSLAQDGETYLMESKDYNLEDQIPEKCEAIASDCFLSGNVDIEKCLQCTLLVIKADKNDECLKYVSKNVKDRFEEILTKGEDDADSDEYDFIAPANYILKNIYKKNDTNGKKELLHFKDINNNLKLELINYCNLLKDNDVSGILTYEKLGNVQDIFNNLTKLLEEHKEENNYVLYHKMKNEVLCLKNANDWMKNKTGLVLPQLKYSLNKFNKNKENYIKENIFEEDENGIVDLTKFPVDTSYSSYNYADSLYCNREYCNRLKDHNNCISKINVEDQKNCALSWAFASIYHLETIKCMKGYEPLNASVLYVTNCLKNKNNDVCTEGSNPLVFLETIEEKGFLPTESNYPYDQSKVGDVCPQVQNDWDNVFENTKVLEYNNAPFSVGTKGYIAYESEVFQKDIDSFVKLIKDEIMNKGSVIAYVKAKNVLGYELNGKKVQNLCGDKKPDHAVNIVGYGNYINNKGEKKSYWIVRNSWGKYWGDDGYFKVDMYGPPTCEDNFIHSVVVFNVEVPVNENFDKKEHDIYKSYLKNSPDFYHNIYYKNYNFENYVSPISTWSEVLHNTLYNNNLIWGQETTDPIGEGKLPASEAGHLRGEGKGNSEENQGQRSNANGAISSNQSTGGKITKQGESKDDGVALPVSTDGKPNTSSSVVDTNDQRSLPNPRATSLQPPSVQIPNHEGTSAPGNSRTPSIVSPTAAEKSRKAQIFHVLKHIKNSRIKMGLVKYDNSDNIGGDHVCSRTYAVNPEKQEECVKFCEENWENCKNKPSPGYCLAKLKNTNECFFCYV

SEQ ID NO: 61 - protein, 930 aa, Plasmodium falciparum
MKFSISLFLILCVLFCKNDIKCTTVDESTKEGSQNPKNSSSTTPASGSQKGSSSESPGSSVEKQSQESNKESTNGGNVVSQGTPANTFGQNSNNPSDSPQGTSTLPSPPKSIDVKSAFLKHYKGVKVTGSCNANFQLFLVPHIFINVETKENNIQLDVKFLKLTKRIDFAKDKSMLKNKCESGKNQTFKFVLYFKDDILTIKWKVYEEKSATPQKSEENTVDIKLYKLPKLDQTITSIQVHTLSIEGTSYLMESKDYSLGNNLPEKCDAIASDCFLSGNINVEKCLKCTLKVKKVEASDECYKYVSKDKPKETKLAVSGSEVKEVKAASVDHSNDKEYELSQSINNILNKMYKKESNDEKNNKKELIKLEDADDSLQKELNKYCNSLKEVDLNGVLSKNEVGNEKDVFNNLTTLLKEHMLESHHVVFEKLKNSALCLKNIDDWLKNKNGLIVPPSKYKLKDTNEKKELNNNVEVIEDMFKANEHGIVDLTKFPIDTNYSSYKHIDHTYCNNDYCNWSKDKNSCISKINVEDQKNCALSWAFASKYHLETIKCMKGYEHIPISSLYIANCSKNEKKDVCTEGSNPLKVLQMIVEKGFLPTEGDYSYEQSKVGETCPEVQNGWVNLWANAKLLEQNNDEHNSLSTKGYTAYESEAFQKDMHSFVKLIKDEIMNKGSVIAYVKADKIMAYEFNGKKVQNLCGDKTPDHAVNIIGYGNYINDEHQKKSYWIVRNSWGKHWGDKGHFKVDMYGPSDCEDNFIHSVVIFNVDLPINQESVKKEPKIYNYYLKASPDFYHNLYYKNFDSQKGKADQAENKKSYLYGQEESTSEQLPSSLSSPQNNKQSERSKEKVDIFHVLKHIKDSKIKMGIVKYDHSDALGEDNVCSRSYSSNPEKQEGCVKFCNENWGKCKDAASPGFCLSELEKTNDCFFCYI

SEQ ID NO: 62 - protein, 962 aa, Plasmodium falciparum
MKIHIFLIATIYVLFSEKLIKWTTASTTQGGDTDTHPGTPPGEGSDVSQGAGQDASQGAGQDANPDPTLPKPPSPPADDTKDTGSQGDADSSSSKIEIPPLVKPENHKTIVSAMLKNYKGVKVTGTCGADFGLFLVPHIYVHVKSEDTEIELSSELAPPEMQTKFDKTQLKKFCVKDDTKKFDFIAYIYKDILVFKWKVYEEGLSKEQDVDEMKYLLPNLKQPITSIQVHSWTGTKESYILESKDYVLGEGMPEKCDAIATDCFLSGFTDIGKCFQCKLLMQEKNINDSCFKYVSSNQKELIKKQLKITAQDDEESSEYHLSESIKNLLKNIYKKNNDDNKKKELLHFENVNSALKSELLNYCNLLKEVNMNGVLKDHQLGNVQDVFNNLTKLLEEHKEENDNVLYHKMKNEALCLKNVNDWMKNKTGLLLPQLSYDLTYKNNNFTEFTQNKSYTSQNIVDKLYCNHEYCNRLKDHNNCISKINVEDQKNCALSWAFASKYHLETIKCMKGYEPLNASVLYVTNCLKNKNKDVCTEGSNPLVFLETIEEKGFLPTESNYPYDQSKVGDICPQLQNDWDNVFENTKVLDYNNGPFSVGTKGYIAYESEAFQKDMHSFVKLVKDEIMNKGSVIAYVKAENVLGYELNGKKVQNLCGDKTPDHVVNIVGYGNYINNKGEKKSYWIVRNSWGKYWGDDGYFKVDMYGPSTCEDNFIHTVVVFNVQVPINEKFDKKEHDIYNYYLKTSPEFYHNLYYKTFNSNKEEKSMNKNSYVYGQDTTPVENEAPRSGVQKPTELSSTESQTVSPPNESQTESLLSGGSQVTNPTLTQSTSSSSGQQETGPLSTQGLSPATGDPKGKEQEASPAEGLSGVLNPTKEVTSEEKIQIIHLLKHIKNSKIRRGLVKYNHEFEVGDNSCSRSTSKNAEMHDECVNICEKYWPECRGTAVPGYCLSTHDDKNECDFCYV

SEQ ID NO: 63 - protein, 997 aa, Plasmodium falciparum
MKSYISLFFILCVIFNKNVIKCTGESQTGNTGGGQAGNTGGDQAGSTGGSPQGSTGASPQGSTGASPQGSTGASQPGSSEPSNPVSSGHSVSTVSVSQTSTSSEKQDTIQVKSALLKDYMGLKVTGPCNENFIMFLVPHIYIDVDTEDTNIELRTTLKKTNNAISFESNSGSLEKKKYVKLPSNGTTGEQGSSTGTVRGDTEPISDSSSSSSSSSSSSSSSSSSSSSSSSSSSESLPANGPDSPTVKPPRNLQNICETGKNFKLVVYIKENTLILKWKVYGETKDTTENNKVDVRKYLINEKETPFTNILIHAYKEHNGTNLIESKNYAIGSDIPEKCDTLASNCFLSGNFNIEKCFQCALLVEKENKNDVCYKYLSEDIVSKFKEIKAETEDDDEDDYTEYKLTESIDNILVKMFKTNENNDKSELIKLEEVDDSLKLELMNYCSLLKDVDTTGTLDNYGMGNEMDIFNNLKRLLIYHSEENINTLKNKFRNAAVCLKNVDDWIVNKRGLVLPELNYDLEYFNEHLYNDKNSPEDKDNKGKGVVHVDTTLEKEDTLSYDNSDNMFCNKEYCNRLKDENNCISNLQVEDQGNCDTSWIFASKYHLETIRCMKGYEPTKISALYVANCYKGEHKDRCDEGSSPMEFLQIIEDYGFLPAESNYPYNYVKVGEQCPKVEDHWMNLWDNGKILHNKNEPNSLDGKGYTAYESERFHDNMDAFVKIIKTEVMNKGSVIAYIKAENVMGYEFSGKKVQNLCGDDTADHAVNIVGYGNYVNSEGEKKSYWIVRNSWGPYWGDEGYFKVDMYGPTHCHFNFIHSVVIFNVDLPMNNKTTKKESKIYDYYLKASPEFYHNLYFKNFNVGKKNLFSEKEDNENNKKLGNNYIIFGQDTAGSGQSGKESNTALESAGTSNEVSERVHVYHILKHIKDGKIRMGMRKYIDTQDVNKKHSCTRSYAFNPENYEKCVNLCNVNWKTCEEKTSPGLCLSKLDTNNECYFCYV

SEQ ID NO: 64 - protein, 1233 aa, Plasmodium falciparum
MRNLFHITICLVTLNLFILEINAKTNTSENRNKRIGGPKLRGNVTSNIKFPSDNKGKIIRGSNDKLNKNSEDVLEQSEKSLVSENVPSGLDIDDIPKESIFIQEDQEGQTHSELNPETSEHSKDLNNNDSKNESSDIISVNNKSNKVQNHFESLSDLELLENSSQDNLDKDTISTEPFPNQKHKDLQQDLNDEPLEPFPTQIHKDYKEKNLINEEDSEPFPRQKHKKVDNHNEEKNVFHENGSANGNQGSLKLKSFDEHLKDEKIENEPLVHENLSIPNDPIEQILNQPEQETNIQEQLYNEKQNVEEKQNSQIPSLDLKEPTNEDILPNHNPLENIKQSESEINHVQDHALPKENIIDKLDNQKEHIDQSQHNINVLQENNINNHQLEPQEKPNIESFEPKNIDSEIILPENVETEEIIDDVPSPKHSNHETFEEETSESEHEEAVSEKNAHETVEHEETVSQESNPEKADNDGNVSQNSNNELNENEFVESEKSEHEPAENEESSLEEGHHEEIVPEQNNEESGESKLVDNDEGGFEEAHHENFSSEVSNSELNENEFVESDKSVTEPAEHEEVVSEESNPEPAENEESSIEEAHQEEIVPEQNDEESGESGLVDNEEGDFEEPNHEEFEPDQNDSELSENELVESEKSVSEPAEHVEIVSEKSVSEPAEHVEIVSEKSTSEPAEHVESVSEQSNNEPSEKKDGPVPSKPFEEIEKVDVQPKIVDLQIIEPNFVDSQPNPQEPVEPSFVKIEKVPSEENKHASVDPEVKEKENVSEVVEEKQNSQESVEEIPVNEDEFEDVHTEQLDLDHKTVDPEIVEVEEIPSELHENEVAHPEIVEIEEVFPEPNQNNEFQEINEDDKSAHIQHEIVEVEEILPEDDKNEKVEHEIVEVEEILPEDKNEKVQHEIVEVEEILPEDKNEKVEHEIVEVEEILPEDKNEKGQHEIVEVEEILPEDKNEKVQHEIVEVEEILPEDKNEKGQHEIVEVEEILPEDKNEKVEHEIVEVEEILPEDKNEKGQHEIVEVEEILPEDDKNEKGQHEIVEVEEILPEIVEIEEVPSQTNNNENIETIKPEEKKNEFSVVEEKAIPQEPVVPTLNENENVTPKPSEGESTKPDIVQIKIVQENKPNKKETPVVDGPKHVEQNIQEDDNDEEDDDDIDFEGLSRKDDEKDSSNKNKKKSSFITYISTKKFKKVSQTIVSVMINAYDGVIQVVSTIKGIAKDIVIFFQNI

SEQ ID NO: 65 - protein, 396 aa, Plasmodium falciparum
DIPKESIFIQEDQEGQTHSELNPETSEHSKDLNNNDSKNESSDIISVNNKSNKVQNHFESLSDLELLENSSQDNLDKDTISTEPFPNQKHKDLQQDLNDEPLEPFPTQIHKDYKEKNLINEEDSEPFPRQKHKKVDNHNEEKNVFHENGSANGNQGSLKLKSFDEHLKDEKIENEPLVHENLSIPNDPIEQILNQPEQETNIQEQLYNEKQNVEEKQNSQIPSLDLKEPTNEDILPNHNPLENIKQSESEINHVQDHALPKENIIDKLDNQKEHIDQSQHNINVLQENNINNHQLEPQEKPNIESFEPKNIDSEIILPENVETEEIIDDVPSPKHSNHETFEEETSESEHEEAVSEKNAHETVEHEETVSQESNPEKADNDGNVSQNSNNELNENE

SEQ ID NO: 66 - protein, 436 aa, Plasmodium falciparum
DGPVPSKPFEEIEKVDVQPKIVDLQIIEPNFVDSQPNPQEPVEPSFVKIEKVPSEENKHASVDPEVKEKENVSEVVEEKQNSQESVEEIPVNEDEFEDVHTEQLDLDHKTVDPEIVEVEEIPSELHENEVAHPEIVEIEEVFPEPNQNNEFQEINEDDKSAHIQHEIVEVEEILPEDDKNEKVEHEIVEVEEILPEDKNEKVQHEIVEVEEILPEDKNEKVEHEIVEVEEILPEDKNEKGQHEIVEVEEILPEDKNEKVQHEIVEVEEILPEDKNEKGQHEIVEVEEILPEDKNEKVEHEIVEVEEILPEDKNEKGQHEIVEVEEILPEDDKNEKGQHEIVEVEEILPEIVEIEEVPSQTNNNENIETIKPEEKKNEFSVVEEKAIPQEPVVPTLNENENVTPKPSEGESTKPDIVQIKIVQENKPNKKETPVVDG

SEQ ID NO: 67 - protein, 824 aa, Plasmodium falciparum
MRLSKVSDIKSTGVSNYKNFNSKNSSKYSLMEVSKKNEKKNSLGAFHSKKILLIFGIIYVVLLNAYICGDKYEKAVDYGFRESRILAEGEDTCARKEKTTLRKSKQKTSTRTVATQTKKDEENKSVVTEEQKVESDSEKQKRTKKVVKKQINIGDTENQKEGKNVKKVIKKEKKKEESGKPEENKHANEASKKQEPKASKVSQKPSTSTRSNNEVKIRAASNQETLTSADPEGQIMREYAADPEYRKHLEIFYKILTNTDPNDEVERRNADNKEDLTSADPEGQIMREYASDPEYRKHLEIFYKILTNTDPNDDVERRNADNKEDLTSADPEGQIMREYAADPEYRKHLEVFHKILTNTDPNDEVERRNADNKEDLTSADPEGQIMREYAADPEYRKHLEVFHKILTNTDPNDEVERRNADNKELTSSDPEGQIMREYAADPEYRKHLEVFHKILTNTDPNDEVERRNADNKEDLTSADPEGQIMREYAADPEYRKHLEVFHKILTNTDPNDEVERRNADNKEDLTSADPEGQIMREYAADPEYRKHLEIFHKILTNTDPNDEVERRNADNKEDLTSADPEGQIMREYAADPEYRKHLEIFYKILTNTDPNDEVERRNADNKEELTSSDPEGQIMREYAADPEYRKHLEIFHKILTNTDPNDEVERRNADNKEDLTSADPEGQIMREYAADPEYRKHLEIFYKILTNTDPNDEVERRNADNKEDLTSADPEGQIMREYASDPEYRKHLEIFYKILTNTDPNDDVERRNADNKEDLTSADPEGQIMREYAADPEYRKHLEVFHKILTNTDPNDEVERQNADNNEA

SEQ ID NO: 68 - protein, 41 aa, Plasmodium falciparum
GMNNMNGDINNINGDINNMNGDINNMNGDINNMNGDINNMN

SEQ ID NO: 69 - protein, 37 aa, Plasmodium falciparum
EEIKEEIKEVKEEIKEVKEEIKEVKEEIKEVKEEIKE

SEQ ID NO: 70 - protein, 28 aa, Plasmodium falciparum
EKLKKYNNEISSLKKELDILNEKMGKCT

SEQ ID NO: 71 - protein, 38 aa, Plasmodium falciparum
TKKLNKELSEGNKELEKLEKNIKELEETNNTLENDIKV

SEQ ID NO: 72 - protein, 526 aa, Plasmodium falciparum
MIRIKKKLILTIIYIHLFILNRLSFENAIKKTKNQENNLTLLPIKSTEEEKDDIKNGKDIKKEIDNDKENIKTNNAKDHSTYIKSYLNTNVNDGLKYLFIPSHNSFIKKYSVFNQINDGMLLNEKNDVKNNEDYKNVDYKNVNFLQYHFKELSNYNIANSIDILQEKEGHLDFVIIPHYTFLDYYKHLSYNSIYHKSSTYGKCIAVDAFIKKINETYDKVKSKCNDIKNDLIATIKKLEHPYDINNKNDDSYRYDISEEIDDKSEETDDETEEVEDSIQDTDSNHTPSNKKKNDLMNRTFKKMMDEYNTKKKKLIKCIKNHENDFNKICMDMKNYGTNLFEQLSCYNNNFCNTNGIRYHYDEYIHKLILSVKSKNLNKDLSDMTNILQQSELLLTNLNKKMGSYIYIDTIKFIHKEMKHIFNRIEYHTKIINDKTKIIQDKIKLNIWRTFQKDELLKRILDMSNEYSLFITSDHLRQMLYNTFYSKEKHLNNIFHHLIYVLQMKFNDVPIKMEYFQTYKKNKPLTQ

SEQ ID NO: 73 - protein, 622 aa, Plasmodium falciparum
MRKLYCVLLLSAFEFTYMINFGRGQNYWEHPYQNSDVYRPINEHREHPKEYEYPLHQEHTYQQEDSGEDENTLQHAYPIDHEGAEPAPQEQNLFSSIEIVERSNYMGNPWTEYMAKYDIEEVHGSGIRVDLGEDAEVAGTQYRLPSGKCPVFGKGIIIENSNTTFLTPVATGNQYLKDGGFAFPPTEPLMSPMTLDEMRHFYKDNKYVKNLDELTLCSRHAGNMIPDNDKNSNYKYPAVYDDKDKKCHILYIAAQENNGPRYCNKDESKRNSMFCFRPAKDISFQNYTYLSKNVVDNWEKVCPRKNLQNAKFGLWVDGNCEDIPHVNEFPAIDLFECNKLVFELSASDQPKQYEQHLTDYEKIKEGFKNKNASMIKSAFLPTGAFKADRYKSHGKGYNWGNYNTETQKCEIFNVKPTCLINNSSYIATTALSHPIEVENNFPCSLYKDEIMKEIERESKRIKLNDNDDEGNKKIIAPRIFISDDKDSLKCPCDPEMVSNSTCRFFVCKCVERRAEVTSNNEVVVKEEYKDEYADIPEHKPTYDKMKIIIASSAAVAVLATILMVYLYKRKGNAEKYDKMDEPQDYGKSNSRNDEMLDPEASFWGEEKRASHTTPVLMEKPYY

SEQ ID NO: 74 - protein, 217 aa, Plasmodium falciparum
MNKLYSLFLFLFIQLSIKYNNAKVTVDTVCKRGFLIQMSGHLECKCENDLVLVNEETCEEKVLKCDEKTVNKPCGDFSKCIKIDGNPVSYACKCNLGYDMVNNVCIPNECKNVTCGNGKCILDTSNPVKTGVCSCNIGKVPNVQDQNKCSKDGETKCSLKCLKENETCKAVDGIYKCDCKDGFIIDNESSICTAFSAYNILNLSIMFILFSVCFFIM

SEQ ID NO: 75 - protein, 2163 aa, Plasmodium falciparum
MVTQSSGGGAAGSSGEEDAKHVLDEFGQQVYNEKVEKYANSKIYKEALKGDLSQASILSELAGTYKPCALEYEYYKHTNGGGKGKRYPCTELGEKVEPRFSDTLGGQCTNKKIEGNKYIKGKDVGACAPYRRLHLCSHNLESIQTNNYNSGNAKHNLLVDVCMAAKYEGDSIKNYYPKYQRTYPDTNSQLCTVLARSFADIGDIVRGKDLYLGNPQESTQRIILENNLKDIFAKIHSDVMSTSGSNGRALQKRYKDTDNYYELREDWWALNRDQVWKAITCNAGGGNRYFRQTCGSGEWAKDKCRCKDDKVPTYFDYVPQYLRWFEEWAEDFCRLRKHKLKDAKNKCRGDSGNDRYCDLNRYDCTQTIRGNEHFVEKDDCKGCQYSCAHFVNWIDNQKLEFEKQKEKYTKEIKKKHPTTIIIKTANRKTTINNLYVKEFYKKLQEKYGDVENFLQKLNEEQICKNQPYNDESSIDINFKSIKDIDIFSHTEYCQACPWCGAKRKGKGWEPKEKTCGKTKTYDPKKTTNIPILTPYISQQSILKKYNKFCNGNGGNGAPATATGGGQIKNWQCHYEGDNNDNCVEGEWKEFKEGKNVMSYNAFFWKWVHDMLIDSMQWRNEHGNCINKDNDNTCKNSCKRPCECFKRWVDQKKKNEWEAIKDHFKKQNIAAETQCDPGVTLQWVLILDFLKDESTEDKENKVSAEEAKEIKHLRQMLQQAGVDDPAAFARPCTEDGVAEQDTIMDKLLNREENDATECKKCDKPPPAPTAGDRGPGARADPHDVQQPRPPGSGPGTDANDEDDDDDDDDDDEEDGEAKEEEEDEEKQEDVHQEEKAKKEEPQKEEVARTPKDDVNVCNIVNNVFTDGSSLQAACSLKYGKNAPTSWKCVTPSGNTSDTTVKSGDTTGGSICVPPRRRRLYVTPLTRLTGGDSTTQASQASEVQTQARGSNTDKSPGSSEAAQGDGVSKDPQKALLKAFVESAAVETFFLWDRYKKIKEKEKKEKKKTYEQIYESTDYDDEEKDPQEELKKGIIPDEFKRQMFYTLGDYKDILYSGDTVNGGNEDKIKKAINNYFQKIREQSSSDNNPSPRSVKTPSTSDKDPQTWWNAHAPSIWNAMVCALTYDTNSGGEGKTTTITQDPNLKTALWDENGKKPLKTKYQYDSVTIGASGAKPQTKAKPTGGDTPLTQFVLRPTYFRYLEEWGQNFCKKRTEMLEKIKYECKVGQGRGGRKQKTPQCSCYGENCDDQLDDNPSTDADLKCPGCGRECRKYKKWIEKKKEEFTKQSNVYEEQKTKCQKESKSAKGNNHGNEFCGTQGTCDTAGDFLNRLKSGPCKKENGKDNQEDEINFKDEDKTFGHENYCAPCPVFKDICKKKDCRNASNNMCNGKDFITAEDIKIMDSSSEEVNMLVSDNDTNKFDGGLDACKDAHIFKGIKENKWSCGNVCGYNVCKPKKVNGEKGSGENNDQIITIRGLVTHWVQNFLDDYNKIRTKLKPCRNNGEVSKCIKDCVKKWVEKKTEEWPKIRDRYLEPYKSDDGYNKKSLVRSFMETLIPLMDLTNGKEKIQELNKFLRSYECNCADNSQQKGDTPKDIVECLLEKLEDKANKCKTQTSGTDCHPSTPLEDDDEPLEETEENTVEQPNICPTKQPQPEKEDGCEAAPTTAEETSPTATSEGTENQSPPPPPPAPAPAPAPAPEKSQPKEDKKVEPQPKPQPTNPPPNLFNNPAVIPALMSSTIMWSIGIGFAAFTYFLLKKKTKSSVGNLFQILQIPQNDYGIPTLKSKNRYIPYRSGTYKGKTYIYMEGDSSGDEKYAFMSDTTDVTSSESEYEELDINDIYVPHAPKYKTLIEVVLEPSGNNTTASGKNTPSDTQNDIPTSDTPPPITDNEWNTLKDEFISQYLQSEQPKDVPNDYKSGDIPLNTQPNTLYFNKPEEKPFITSIHDRDLYTGEQISYNIHMSTNTMDDPKYVSNNVYSGIDLINDALNGDYDIYDEILKRKENELFGTNHVKQTSIHSVAKLTNSDPIHNQLELFHKWLDRHRNMCEKWKNDNERLAKLKEEWENETHSGNTHPSDSNKTLNTDVSIQIDMDHEKRMKEFTNMDTILDDLKTYNEPYYDVQDDIYYDVNDHDASTVDSNNMDVPSRVQIEMDVNTKLVKEKYPIADVWDI

SEQ ID NO: 76 - protein, 1558 aa, Plasmodium falciparum
MTNSNYKSNNKTYNENNNEQITTIFNRTNMNPIKKCHMREKINKYFFLIKILTCTILIWAVQYANNSDINKSWKKNTYVDKKLNKLFNRSLGESQVNGELASEEVKEKILDLLEEGNTLTESVDDNKNLEEAEDIKENILLSNIEEPKENIIDNLLNNIGQNSEKQESVSENVQVSDELFNELLNSVDVNGEVKENILEESQVNDDIFNSLVKSVQQEQQHNVEEKVEESVEENDEESVEENVEENVEENDDESVASSVEESIASSVDESIDSSIEENVAPTVEEIVAPTVEEIVAPSVVESVAPSVEESVEENVEESVAENVEESVAENVEESVAENVEESVAENVEESVAENVEESVAENVEEIVAPTVEESVAPTVEEIVAPSVEESVAPSVEEIVVPTVEESVAENVEEIVAPSVEEIVAPSVEEIVAPTVEESVAPTVEEIVAPSVEESVAPSVEEIVVPTVEESVAENVEESVAENVEEIVAPSVEEIVAPSVEEIVAPSVEEIVAPSVEEIVAPSVEEIVAPSVEEIVAPSVEEIVAPSVEEIVAPTVEEIVAPTVEEIVAPSVEEIVAPTVEESVAENVATNLSDNLLSNLLGGIETEEIKDSILNEIEEVKENVVTTILENVEETTAESVTTFSNILEEIQENTITNDTIEEKLEELHENVLSAALENTQSEEEKKEVIDVIEEVKEEVATTLIETVEQAEEESASTITEIFENLEENAVESNENVAENLEKLNETVFNTVLDKVEETVEISGESLENNEMDKAFFSEIFDNVKGIQENLLTGMFRSIETSIVIQSEEKVDLNENVVSSILDNIENMKEGLLNKLENISSTEGVQETVTEHVEQNVYVDVDVPAMKDQFLGILNEAGGLKEMFFNLEDVFKSESDVITVEEIKDEPVQKEVEKETVSIIEEMEENIVDVLEEEKEDLTDKMIDAVEESIEISSDSKEETESIKDKEKDVSLVVEEVQDNDMDESVEKVLELKNMEEELMKDAVEINDITSKLIEETQELNEVEADLIKDMEKLKELEKALSEDSKEIIDAKDDTLEKVIEEEHDITTTLDEVVELKDVEEDKIEKVSDLKDLEEDILKEVKEIKELESEILEDYKELKTIETDILEEKKEIEKDHFEKFEEEAEEIKDLEADILKEVSSLEVEEEKKLEEVHELKEEVEHIISGDAHIKGLEEDDLEEVDDLKGSILDMLKGDMELGDMDKESLEDVTAKLGERVESLKDVLSSALGMDEEQMKTRKKAQRPKLEEVLLKEEVKEEPKKKITKKKVRFDIKDKEPKDEIVEVEMKDEDIDEDIEEDVEEDIEEDKVEDIDEDIDEDIDEDIGEDKDEVIDLIVQKEKRIEKVKEKKKKLEKKVEEGVSGLKKHVDEVMKYVQKIDKEVDKEVSKALESKNDVTNVLKQNQDFFSKVKNFVKKYKVFAAPFISAVAAFASYVVGFFTFSLFSSCVTIASSTYLLSKVDKTINKNKERPFYSFVFDIFKNLKHYLQQMKEKFSKEKNNNVIEVTNKAEKKGNVQVTNKTEKTTKVDKNNKVPKKSRTQKSK

SEQ ID NO: 77 - protein, 150 aa, Plasmodium falciparum
SDELFNELLNSVDVNGEVKENILEESQVNDDIFNSLVKSVQQEQQHNVEEKVEESVEENDEESVEENVEENVEENDDESVASSVEESIASSVDESIDSSIEENVAPTVEEIVAPTVEEIVAPSVVESVAPSVEESVEENVEESVAENVEE

SEQ ID NO: 78 - protein, 397 aa, Plasmodium falciparum
MMRKLAILSVSSFLFVEALFQEYQCYGSSSNTRVLNELNYDNAGTNLYNELEMNYYGKQENWYSLKKNSRSLGENDDGNNEDNEKLRKPKHKKLKQPADGNPDPNANPNVDPNANPNVDPNANPNVDPNANPNANPNANPNANPNANPNANPNANPNANPNANPNANPNANPNANPNANPNANPNANPNANPNANPNVDPNANPNANPNANPNANPNANPNANPNANPNANPNANPNANPNANPNANPNANPNANPNANPNANPNANPNANPNKNNQGNGQGHNMPNDPNRNVDENANANSAVKNNNNEEPSDKHIKEYLNKIQNSLSTEWSPCSVTCGNGIQVRIKPGSANKPKDELDYANDIEKKICKMEKCSSVFNVVNSSIGLIMVLSFLFLN

SEQ ID NO: 79 - protein, 574 aa, Plasmodium falciparum
MNHLGNVKYLVIVFLIFFDLFLVNGRDVQNNIVDEIKYREEVCNDEVDLYLLMDCSGSIRRHNWVNHAVPLAMKLIQQLNLNDNAIHLYASVFSNNAREIIRLHSDASKNKEKALIIIKSLLSTNLPYGKTNLTDALLQVRKHLNDRINRENANQLVVILTDGIPDSIQDSLKESRKLSDRGVKIAVFGIGQGINVAFNRFLVGCHPSDGKCNLYADSAWENVKNVIGPFMKAVCVEVEKTASCGVWDEWSPCSVTCGKGTRSRKREILHEGCTSELQEQCEEERCLPKREPLDVPDEPEDDQPRPRGDNFAVEKPNENIIDNNPQEPSPNPEEGKGENPNGFDLDENPENPPNPPNPPNPPNPPNPPNPDIPEQEPNIPEDSEKEVPSDVPKNPEDDREENFDIPKKPENKHDNQNNLPNDKSDRYIPYSPLSPKVLDNERKQSDPQSQDNNGNRHVPNSEDRETRPHGRNNENRSYNRKHNNTPKHPEREEHEKPDNNKKKAGSDNKYKIAGGIAGGLALLACAGLAYKFVVPGAATPYAGEPAPFDETLGEEDKDLDEPEQFRLPEENEWN

SEQ ID NO: 80 - protein, 272 aa, Plasmodium falciparum; identical to SEQ ID NO: 55

SEQ ID NO: 81 - protein, 560 aa, Plasmodium falciparum
MSRKLFASILIGALLGIGAPPSAHAGADDVVDSSKSFVMENFSSYHGTKPGYVDSIQKGIQKPKSGTQGNYDDDWKGFYSTDNKYDAAGYSVDNENPLSGKAGGVVKVTYPGLTKVLALKVDNAETIKKELGLSLTEPLMEQVGTEEFIKRFGDGASRVVLSLPFAEGSSSVEYINNWEQAKALSVELEINFETRGKRGQDAMYEYMAQACAGNRVRRSVGSSLSCINLDWDVIRDKTKTKIESLKEHGPIKNKMSESPNKTVSEEKAKQYLEEFHQTALEHPELSELKTVTGTNPVFAGANYAAWAVNVAQVIDSETADNLEKTTAALSILPGIGSVMGIADGAVHHNTEEIVAQSIALSSLMVAQAIPLVGELVDIGFAAYNFVESIINLFQVVHNSYNRPAYSPGHKTQPFLHDGYAVSWNTVEDSIIRTGFQGESGHDIKITAENTPLPIAGVLLPTIPGKLDVNKSKTHISVNGRKIRMRCRAIDGDVTFCRPKSPVYVGNGVHANLHVAFHRSSSEKIHSNEISSDSIGVLGYQKTVDHTKVNSKLSLFFEIKS

SEQ ID NO: 82 - protein, 535 aa, Plasmodium falciparum
GADDVVDSSKSFVMENFSSYHGTKPGYVDSIQKGIQKPKSGTQGNYDDDWKEFYSTDNKYDAAGYSVDNENPLSGKAGGVVKVTYPGLTKVLALKVDNAETIKKELGLSLTEPLMEQVGTEEFIKRFGDGASRVVLSLPFAEGSSSVEYINNWEQAKALSVELEINFETRGKRGQDAMYEYMAQACAGNRVRRSVGSSLSCINLDWDVIRDKTKTKIESLKEHGPIKNKMSESPNKTVSEEKAKQYLEEFHQTALEHPELSELKTVTGTNPVFAGANYAAWAVNVAQVIDSETADNLEKTTAALSILPGIGSVMGIADGAVHHNTEEIVAQSIALSSLMVAQAIPLVGELVDIGFAAYNFVESIINLFQVVHNSYNRPAYSPGHKTQPFLHDGYAVSWNTVEDSIIRTGFQGESGHDIKITAENTPLPIAGVLLPTIPGKLDVNKSKTHISVNGRKIRMRCRAIDGDVTFCRPKSPVYVGNGVHANLHVAFHRSSSEKIHSNEISSDSIGVLGYQKTVDHTKVNSKLSLFFEIKS

SEQ ID NO: 83 - protein, 1315 aa, Plasmodium falciparum
MPITINNFRYSDPVNNDTIIMMEPPYCKGLDIYYKAFKITDRIWIVPERYEFGTKPEDFNPPSSLIEGASEYYDPNYLRTDSDKDRFLQTMVKLFNRIKNNVAGEALLDKIINAIPYLGNSYSLLDKFDTNSNSVSFNLLEQDPSGATTKSAMLTNLIIFGPGPVLNKNEVRGIVLRVDNKNYFPCRDGFGSIMQMAFCPEYVPTFDNVIENITSLTIGKSKYFQDPALLLMHELIHVLHGLYGMQVSSHEIIPSKQEIYMQHTYPISAEELFTFGGQDANLISIDIKNDLYEKTLNDYKAIANKLSQVTSCNDPNIDIDSYKQIYQQKYQFDKDSNGQYIVNEDKFQILYNSIMYGFTEIELGKKFNIKTRLSYFSMNHDPVKIPNLLDDTIYNDTEGFNIESKDLKSEYKGQNMRVNTNAFRNVDGSGLVSKLIGLCKKIIPPTNIRENLYNRTASLTDLGGELCIKIKNEDLTFIAEKNSFSEEPFQDEIVSYNTKNKPLNFNYSLDKIIVDYNLQSKITLPNDRTTPVTKGIPYAPEYKSNAASTIEIHNIDDNTIYQYLYAQKSPTTLQRITMTNSVDDALINSTKIYSYFPSVISKVNQGAQGILFLQWVRDIIDDFTNESSQKTTIDKISDVSTIVPYIGPALNIVKQGYEGNFIGALETTGVVLLLEYIPEITLPVIAALSIAESSTQKEKIIKTIDNFLEKRYEKWIEVYKLVKAKWLGTVNTQFQKRSYQMYRSLEYQVDAIKKIIDYEYKIYSGPDKEQIADEINNLKNKLEEKANKAMININIFMRESSRSFLVNQMINEAKKQLLEFDTQSKNILMQYIKANSKFIGITELKKLESKINKVFSTPIPFSYSKNLDCWVDNEEDIDVILKKSTILNLDINNDIISDISGFNSSVITYPDAQLVPGINGKAIHLVNNESSEVIVHKAMDIEYNDMFNNFTVSFWLRVPKVSASHLEQYGTNEYSIISSMKKHSLSIGSGWSVSLKGNNLIWTLKDSAGEVRQITFRDLPDKFNAYLANKWVFITITNDRLSSANLYINGVLMGSAEITGLGAIREDNNITLKLDRCNNNNQYVSIDKFRIFCKALNPKEIEKLYTSYLSITFLRDFWGNPLRYDTEYYLIPVASSSKDVQLKNITDYMYLTNAPSYTNGKLNIYYRRLYNGLKFIIKRYTPNNEIDSFVKSGDFIKLYVSYNNNEHIVGYPKDGNAFNNLDRILRVGYNAPGIPLYKKMEAVKLRDLKTYSVQLKLYDDKNASLGLVGTHNGQIGNDPNRDILIASNWYFNHLKDKILGCDWYFVPTDEGWTND

SEQ ID NO: 84 - protein, 364 aa, Plasmodium falciparum
MKLKTLALSLLAAGVLAGCSSHSSNMANTQMKSDKIIIAHRGASGYLPEHTLESKALAFAQQADYLEQDLAMTKDGRLVVIHDHFLDGLTDVAKKFPHRHRKDGRYYVIDFTLKEIQSLEMTENFETKDGKQAQVYPNRFPLWKSHFRIHTFEDEIEFIQGLEKSTGKKVGIYPEIKAPWFHHQNGKDIAAETLKVLKKYGYDKKTDMVYLQTFDFNELKRIKTELLPQMGMDLKLVQLIAYTDWKETQEKDPKGYWVNYNYDWMFKPGAMAEVVKYADGVGPGWYMLVNKEESKPDNIVYTPLVKELAQYNVEVHPYTVRKDALPAFFTDVNQMYDALLNKSGATGVFTDFPDTGVEFLKGIK

SEQ ID NO: 85 - protein, 757 aa, synthetic construct
  REGION 1..757: note = PP21 biofusion protein
MKYLLPTAAAGLLLLAAQPAMAMGKTKEYAEKAKNAYEKAKNAYQKANQAVLKAKEASSYDYILGWEFGGGVPEHKKEENMLSHLYVSSKDKENISKENDDVLDEKEEEAEETEEEELEGADDVVDSSKSFVMENFSSYHGTKPGYVDSIQKGIQKPKSGTQGNYDDDWKEFYSTDNKYDAAGYSVDNENPLSGKAGGVVKVTYPGLTKVLALKVDNAETIKKELGLSLTEPLMEQVGTEEFIKRFGDGASRVVLSLPFAEGSSSVEYINNWEQAKALSVELEINFETRGKRGQDAMYEYMAQACAGNRVRRSVGSSLSCINLDWDVIRDKTKTKIESLKEHGPIKNKMSESPNKTVSEEKAKQYLEEFHQTALEHPELSELKTVTGTNPVFAGANYAAWAVNVAQVIDSETADNLEKTTAALSILPGIGSVMGIADGAVHHNTEEIVAQSIALSSLMVAQAIPLVGELVDIGFAAYNFVESIINLFQVVHNSYNRPAYSPGHKTQPFLHDGYAVSWNTVEDSIIRTGFQGESGHDIKITAENTPLPIAGVLLPTIPGKLDVNKSKTHISVNGRKIRMRCRAIDGDVTFCRPKSPVYVGNGVHANLHVAFHRSSSEKIHSNEISSDSIGVLGYQKTVDHTKVNSKLSLFFEIKSKTKEYAEKAKNAYEKAKNAYQKANQAVLKAKEASSYDYILGWEFGGGVPEHKKEENMLSHLYVSSKDKENISKENDDVLDEKEEEAEETEEEELELEHHHHHH

SEQ ID NO: 86 - protein, 727 aa, synthetic construct
  REGION 1..727: note = PP22 biofusion protein
MKYLLPTAAAGLLLLAAQPAMAMGLNNNILGWEFGGGAPQNGAAEDKKTEYLLEQIKIPSWDRNNIPDENEQVIEDPQEDNKDEDEDEETETENLETEDDNNEEGADDVVDSSKSFVMENFSSYHGTKPGYVDSIQKGIQKPKSGTQGNYDDDWKEFYSTDNKYDAAGYSVDNENPLSGKAGGVVKVTYPGLTKVLALKVDNAETIKKELGLSLTEPLMEQVGTEEFIKRFGDGASRVVLSLPFAEGSSSVEYINNWEQAKALSVELEINFETRGKRGQDAMYEYMAQACAGNRVRRSVGSSLSCINLDWDVIRDKTKTKIESLKEHGPIKNKMSESPNKTVSEEKAKQYLEEFHQTALEHPELSELKTVTGTNPVFAGANYAAWAVNVAQVIDSETADNLEKTTAALSILPGIGSVMGIADGAVHHNTEEIVAQSIALSSLMVAQAIPLVGELVDIGFAAYNFVESIINLFQVVHNSYNRPAYSPGHKTQPFLHDGYAVSWNTVEDSIIRTGFQGESGHDIKITAENTPLPIAGVLLPTIPGKLDVNKSKTHISVNGRKIRMRCRAIDGDVTFCRPKSPVYVGNGVHANLHVAFHRSSSEKIHSNEISSDSIGVLGYQKTVDHTKVNSKLSLFFEIKSLNNNILGWEFGGGAPQNGAAEDKKTEYLLEQIKIPSWDRNNIPDENEQVIEDPQEDNKDEDEDEETETENLETEDDNNEELEHHHHHH

SEQ ID NO: 87 - protein, 709 aa, synthetic construct
  REGION 1..709: note = PP23 biofusion protein
MKYLLPTAAAGLLLLAAQPAMAMGLNNNILGWEFGGGAPQNGAAEDKKTEYLLEQIKIPSWDRNNIPDENEQVIEDPQEDNKDEDEDEETETENLETEDDNNEEGADDVVDSSKSFVMENFSSYHGTKPGYVDSIQKGIQKPKSGTQGNYDDDWKEFYSTDNKYDAAGYSVDNENPLSGKAGGVVKVTYPGLTKVLALKVDNAETIKKELGLSLTEPLMEQVGTEEFIKRFGDGASRVVLSLPFAEGSSSVEYINNWEQAKALSVELEINFETRGKRGQDAMYEYMAQACAGNRVRRSVGSSLSCINLDWDVIRDKTKTKIESLKEHGPIKNKMSESPNKTVSEEKAKQYLEEFHQTALEHPELSELKTVTGTNPVFAGANYAAWAVNVAQVIDSETADNLEKTTAALSILPGIGSVMGIADGAVHHNTEEIVAQSIALSSLMVAQAIPLVGELVDIGFAAYNFVESIINLFQVVHNSYNRPAYSPGHKTQPFLHDGYAVSWNTVEDSIIRTGFQGESGHDIKITAENTPLPIAGVLLPTIPGKLDVNKSKTHISVNGRKIRMRCRAIDGDVTFCRPKSPVYVGNGVHANLHVAFHRSSSEKIHSNEISSDSIGVLGYQKTVDHTKVNSKLSLFFEIKSSNEKGRPPTYSPILDDGIEFSGGLYFNEKKSTEENKQKNVLESVNLTSWDKEDIVKENEDVKLEHHHHHH

SEQ ID NO: 88 - protein, 867 aa, synthetic construct
  REGION 1..867: note = PP25 biofusion protein
MKYLLPTAAAGLLLLAAQPAMAMGSDELFNELLNSVDVNGEVKENILEESQVNDDIFNSLVKSVQQEQQHNVEEKVEESVEENDEESVEENVEENVEENDDESVASSVEESIASSVDESIDSSIEENVAPTVEEIVAPTVEEIVAPSVVESVAPSVEESVEENVEESVAENVEEGADDVVDSSKSFVMENFSSYHGTKPGYVDSIQKGIQKPKSGTQGNYDDDWKEFYSTDNKYDAAGYSVDNENPLSGKAGGVVKVTYPGLTKVLALKVDNAETIKKELGLSLTEPLMEQVGTEEFIKRFGDGASRVVLSLPFAEGSSSVEYINNWEQAKALSVELEINFETRGKRGQDAMYEYMAQACAGNRVRRSVGSSLSCINLDWDVIRDKTKTKIESLKEHGPIKNKMSESPNKTVSEEKAKQYLEEFHQTALEHPELSELKTVTGTNPVFAGANYAAWAVNVAQVIDSETADNLEKTTAALSILPGIGSVMGIADGAVHHNTEEIVAQSIALSSLMVAQAIPLVGELVDIGFAAYNFVESIINLFQVVHNSYNRPAYSPGHKTQPFLHDGYAVSWNTVEDSIIRTGFQGESGHDIKITAENTPLPIAGVLLPTIPGKLDVNKSKTHISVNGRKIRMRCRAIDGDVTFCRPKSPVYVGNGVHANLHVAFHRSSSEKIHSNEISSDSIGVLGYQKTVDHTKVNSKLSLFFEIKSSDELFNELLNSVDVNGEVKENILEESQVNDDIFNSLVKSVQQEQQHNVEEKVEESVEENDEESVEENVEENVEENDDESVASSVEESIASSVDESIDSSIEENVAPTVEEIVAPTVEEIVAPSVVESVAPSVEESVEENVEESVAENVEELEHHHHHH

SEQ ID NO: 89 - protein, 807 aa, Plasmodium falciparum
IPEEQIEEVIQEEIIEQVVPEELIEEVVPEEIIEEVIPEEIVEEVIYEEVIPEELVEEVIAEKLVKEIVPEQVREEVTLEEIVEEMIPEEFVEEVAPEVEIEEIIPEELIEEVIPEVLVEEAVPEELIEKVIPGADDVVDSSKSFVMENFSSYHGTKPGYVDSIQKGIQKPKSGTQGNYDDDWKEFYSTDNKYDAAGYSVDNENPLSGKAGGVVKVTYPGLTKVLALKVDNAETIKKELGLSLTEPLMEQVGTEEFIKRFGDGASRVVLSLPFAEGSSSVEYINNWEQAKALSVELEINFETRGKRGQDAMYEYMAQACAGNRVRRSVGSSLSCINLDWDVIRDKTKTKIESLKEHGPIKNKMSESPNKTVSEEKAKQYLEEFHQTALEHPELSELKTVTGTNPVFAGANYAAWAVNVAQVIDSETADNLEKTTAALSILPGIGSVMGIADGAVHHNTEEIVAQSIALSSLMVAQAIPLVGELVDIGFAAYNFVESIINLFQVVHNSYNRPAYSPGHKTQPFLHDGYAVSWNTVEDSIIRTGFQGESGHDIKITAENTPLPIAGVLLPTIPGKLDVNKSKTHISVNGRKIRMRCRAIDGDVTFCRPKSPVYVGNGVHANLHVAFHRSSSEKIHSNEISSDSIGVLGYQKTVDHTKVNSKLSLFFEIKSIPEEQIEEVIQEEIIEQVVPEELIEEVVPEEIIEEVIPEEIVEEVIYEEVIPEELVEEVIAEKLVKEIVPEQVREEVTLEEIVEEMIPEEFVEEVAPEVEIEEIIPEELIEEVIPEVLVEEAVPEELIEKVIPHHHHHH